European Patent Specification EP 4 062 774 B1, published March 20, 2024. Title: Composition and Methods for Producing Tobacco Plants and Products Having Increased Phenylalanine and Reduced Tobacco-Specific Nitrosamines (TSNAs). Applicant: Altria Client Services LLC. Application EP Div of EP19717695.1. The sequence listing filed with the application follows.

SEQUENCE LISTING (73 sequences)

SEQ ID NO: 1 - protein, 330 aa, Nicotiana
MESKSSGGGEGKVVCVTGASGFIASWLVKMLLQRGYTVNATVRNLKDASKVDHLLGLDGAKERLHLFKAELLGEHSFDPAVDGCEGVFHTASPVSLTAKSKEELVDPAVSGTLNVLRSCTKSTSVRRVVITSSTASVICNKNMSTPGAVADETWYSDAELCEERKEWYQLSKTLAEEAAWKFAKENGLDLVTLHPGLVIGPLLQPTLNFSCEAIVNFIKEGKEAWSGGIYRFVDVRDVANAHILAFEVPSANGRYCLVGVNGYSSLVLKIVQKLYPSITLPENFEDGLPLIPTFQVSSERAKSLGVNFTSLELSVKDTVESLIEKNFLKI

SEQ ID NO: 2 - protein, 416 aa, Nicotiana
MMCNIISLVSIINFFLLFYRVVVLPQHAAASHSTVEFLPGFEGPLPFHLETGYIGVGEYEEVQLFYYFLKSESEPTKDPILIWLSGGPGCSSFTALVYQIGPLYFEPNEYNGSLPKLTLNPNSWTKVANIIFLDQPVNSGFSYATTSTTFKSTDLQACHHIYQFLRKWLIKHQEFIRNPMYIGGDSYSGITVPVITQLISNGIEAGHKPSINLKGYILGNPSTFPLQYNYWVPYAHGMGLISDELYQATTLILYFKIYHIINAINLAYMVEVHRLSTYWANDPRVQEALNVRKGAITRWTRCRESIVNKTYTITFQDSIPYHVELSKKLYRSLIYSGDHDMGIPFQSTQFWIKSLNYSIVDEWRPWSFDGQVAGYTRSYSNQMTFATVKGAGHVAPEYKPKECFTMFQRWLSHEPL

SEQ ID NO: 3 - protein, 569 aa, Nicotiana
MLSVASVEAQKAELSSSVIPPSDQSTEEIHVFRSRLPDIQISNNVPLHVYLFERLSEFQDRTCLIAGSSGQSYTFAETHLICQKIAAGLTNIGIKKGDVIMTFLQNCAEFVFTFLSASMIGAVITTANPFYTKAEAFKQLKASNAKLIVTQSQYVDKFRDSGENDPKIGEDFSVITIDDPPENCLHFSVLSEANEEEMPKGIVIQPDDPVALPFSSGTTGLPKGVILTHKSLITGVAQLVDGDNPNLYLKQDDVVLCVLPLFHIFALNSVLLVSLRAGASVLLMQKFEIGALLELIQNHRVSVAAVVPPLVLALAKNPMVDSFDLSSIRLVLSGAAPLGKELEEALHQRVPQAIFGQGYGMTEAGPVVTMCPAFAKQPFSTKSGSCGSVVRNADLKVVDPETGGSLGRNQPGEICIRGSQIMKGYLNDDEATARTIDVDGWLHTGDIGYVDDDDEIYIVDRVKELIKFKGFQVPPAELESLLVSHPDIADAAVVPQKDDAAGEVPVAFVVRSANGFEITEEAIKEFIAKQVIFYKRLHKVYFIHAIPKSPSGKILRKELRAKLAAPSTQ

SEQ ID NO: 4 - protein, 551 aa, Nicotiana
MGTRAVESSQQQECEHIFRSRYPPVQVPDNVTLPDFVLHNVELYTDKMAFVDATTGKGYTYGQVARDIRRFAKALRSLGLRKGRVVVVVLPNVPEYAIVALGIMAAGGVFSGANPAAHSSEIVKQVESADGKLIVSDLPTYHKVKDCGLPVIILGEEHVEGTIHWDELLEAAERAGSRTDHITNHEDEMVQQNDLCALPFSSGTTGLSKGVMLTHRNLVANLCSTLFSVSPEMVGQVTTLGLIPFFHIYGITGICCATIRNKGKVVVLRRYELRAFLNALITHEVTFAPIVPPIILALVKNPIVDEFDLSKLKLRSIMTAAAPLAPEILNEFEKKFPDVQVQEAYGMTEHSCITLSHSDQHTAKRNSVGFILPNLEVKFVDPDTGRSLPKNKPGEICVKSQCVMKGYYKNEFETCLTIDKDGWLQTGDIGYIDDDGDIFLVDRIKELIKYKGFQVAPAELEGILLTHPSVEDAAVVGLPDEEAGEIPVAWVVLNSKAKESEEDIINYIASTVAQYKRVRVVQFVDSIPKSPSGKILRRLIKDKMLERLKNA

SEQ ID NO: 5 - protein, 671 aa, Nicotiana
MTEIPPNSQMKTMLQKAVQSVQWTYTLFWQLCPQQGALVWRDGYYNGAIKTRKTVQPMEVSAEEASLHRSQQLRELYESLSAGESNQPARRPSAALSPEDLTESEWFYLMCVSFSFPPGIGLPGKAYSKKHHIWIMGANEVDSKVFCRAILAKSARIQTVVGIPLLDGVLELGTTERVQEEIGFINHVKSFFTEQQQPQLPKPALSEHSTSNPTTFSEPHFYSGNTSPSANVDIAHQDGGAAGEEDEEEEEEEDDDEAELDSDSIAIQSAANPIAVEASELMQLDVSEAIQLGSPDDDSDNMDSDFHLVGAGNTAHDYQRQADSFKAETAISWPHFQDLQQLPGGSSYDELSQEDTHYSQTVSTILEHRSSKFSSTTMGCISHDSAQSAFTLCPSTTVCSPNPAHCRHDDSLVDGGGASQWLLKSILFTVPFLHTKYQSEASPKSRDVATVDSSSTASRFRKGCSITSQEEPSGNHVLAERRRREKLNERFIILRSLVPFVTKMDKASILGDTIEYVKQLRKKVQDLEARARDTEHSRDADKKGGTATVKVLQGRGKRRMNTVDGSVGGGQATITASPPSTTENEEVVQVQVSIIESDALVELRCPYKEGLLLNVMQMLRELKVEVVAIQSALNNGVFLAELRAKVKENICGRKASILEVKRSIHQIIPRD

SEQ ID NO: 6 - protein, 683 aa, Nicotiana
MTEIPPNSQMQTMLQKAVQSVQWTYTLFWQLCSQQGVLVWRDGYYNGAIKTRKTVQPMEVSAEEASLHRSQQLRELYESLSAGESNQPARRPSAALSPEDLTESEWFYLMCVSFSFPPGIGLPGKAYSKKHHIWIMCANEVDSKVFCRAILAKSARIQTVVCIPLLDGVLELGTTERVQEDIGFINHVKSFFTEQQQPQPPKPALSEHSTSNSTTFSEPHFYSGNTPPSGNADIAQQDGGAAGEEDEEEEEEEDDEAELDSDSIAIQSEVGGAANPIAAEASELMQLDMSEAIRLGSPDDGSNNMDSDFHLVGAGNTADYQRQPDSFKAETAISWAHFQDLQHLPGGSSYEELSQEDTHYSQTVSTILEHFSNRSSKFSSTTMGCISHDSAQSAFTLCPSTTVDCSPNPAHCRRRHDDSLLDGGGASPSSQWLLKSILFTVPFLHTKYQSEASPKSVDVATVDSSSTASRFRKGCSITSQEEPSGNHVLAERRRREKLNERFIILRSLVPFVTKMDKASILGDTIEYVKQLHKKVQDLEARARHTEQSKDADQKSGTATVKVLQGRGKRRMNTVEAGNIGGGQAKMTAFPLSTTEDEEVVQVEVSIIESDALLELRCPYKEGLLLDVMQMLRELKVEVVAIQSSLNNGIFLAELRAKVKENIYGRKASIVEVKKSIHQIIPRD

SEQ ID NO: 7 - protein, 220 aa, Nicotiana
MNICTNKSSSGVKKGAWTEEEDVLLKKCIEKYGEGKWHQVPLRAGLNRCRKSCRLRWLNYLRPHIKRGDFSFDEVDLILRLHKLLGNRWSLIAGRLPGRTANDVKNYWNSHLRKKLIAPHDQKESKQKAKKITIFRPRPRTFSKTNTCVKSNTNTVDKDIEGSSEIIRFNDNLKPTTEELTDDGIQWWADLLANNYNNNGIEEADNSSPTLLHEEMPLLS

SEQ ID NO: 8 - protein, 419 aa, Nicotiana
MVVISAVVPTPSRVESLAKSGIQAIPKEYVRPQEELNGIGNIFEEEKKDEGPQVPTIDLKEIDSEDKEIREKCHKELKKAAMEWGVMYLVNHGISDQLIDRVKVAGKTFFDQPVEEKEKYANDQPSGNVQGYGSKLANSACGQLEWEDYFFHCVFPEDKCDLSIWPKIPTDYIPATSEYAKQIRNLATKILAVLSIGLGLEEGRLEKEVGGKEDLLLQMKINYYPKCPQPELALGVEAHTDVSALTFILHNMVPGLQLFYEGQWVTAKCVPNSIIMHIGDTLEILSNGKYKSILHRGVVNKEKVRISWAIFCEPPKEKIILKPLSETITEAEPPRFPPRTFAQHMAHKLFKKDDQDAAAEHKVSKKDDPDSAAGHKPFKKDDQDAVVQQKVLKEDEQDAAAEHKVFKKDNQDAAAEESK

SEQ ID NO: 9 - protein, 419 aa, Nicotiana
MVVISAVVPTPSRVESLAKSGIQAIPKEYVRPQEELNGIGNIFEEEKKDEGPQVPTIDLTEIDSEDKEIREKCHQELKKAAIEWGVMHLVNHGISDELIDRVKVSGDTFFDQPVEEKEKYANDQPSGNVQGYGSKLANSACGQLEWEDYFFHCVFPEDKCNLSIWPKTPTDYIPATSEYAKQIRNLATKILAVLSIGLRLEEGRLEKEVGGMEDLLLQMKINYYPKCPQPELALGVEAHTDVSALTFILHNMVPGLQLFYEGQWVTAKCVPNSIIMHIGDTLEILSNGKYKSILHRGVVNKEKIRISWAIFCEPPKEKIILKPLPETITEAEPPRFPPRTFAQHMAHKLFKKDDQDAAAEHKVSKKDDPDSAAEHKPFKKDDQDAVAQQKVLKEDEQNAAAEHKVFKKDNQDAAAEESK

SEQ ID NO: 10 - protein, 622 aa, Nicotiana
MAMGHQDQDGVPNNLRKQLALAVRGIQWSYAIFWSTPVTQPGVLEWSDGYYNGDIKTRKTVQVGEVNEDQLGLHRTEQLRELYSSLLTGEGEEDLQPQAKRPSAALSPEDLTDTEWYFLVCMSFVFNVGQGLPGKTSATNQTIWLCNAHQAESRVFSRSLLAKSASIQTVVCFPYLGGVIELGVTELVLEDPNLIQQIKNSFEVDHSVISKRPNYNSNDAKDDMNVASRKLDHNVLESDAYPVEINNSSPHDSSNGFVANQEAEDSLMVVGVIGETSQAQSWKFVDDNMSNGVHNSLNSSDCISQNYEKLSPLSNGEKETKPCPIDRQEHNQNKLHLLDHQGDDAQYQAVISTLLKSSDQLTLGPHFRNINKKSSFAGWKNDTEAPRIGTAQKLLKKVLLEVPRMHGGVTHKFSRENRKKNGLWRPEVDDIDRSRVISERRRREKINERFMHLASMLPTGGKVDKISLLDETIEYMKELERRVQELEARSGKKTNDTAEQTSDNCGTSKFNDVNGSLKRKACDMDEMEPESCNELLKGSSADGIVISMIDKEVSIKMRCLWSEGLLLKIMEALTDLQMDCHTVQSSKIDGILSIAIESKSNGLKTVSVGAIREVLQRVVWKS

SEQ ID NO: 11 - protein, 364 aa, Nicotiana
MESSTKSQIPTQSEEERNCTYAMQLLSSSVLPFVLHSTIQLEVFEILAKSNDTKLSASQIVSQIPNCTKPEAPTMLNRMLYVLASYSLFTCSIVEDEKNNGGQKRVYGLSQVGKFFVKNENGASMGPLLALLQNKVFINSWFELKDAVLEGGVPFDRVHGVHAFEYPKSDPKFNDVFNKAMINHTTVVMKKILENYKGFENLKTLVDVGGGLGVNLKMITSKYPTIKGTNFDLPHVVQHAPSYPGVEHVGGDMFESVPEGDAIFMKWILHDWSDSHNLKLLKNCYKALPDNGKVIVVEAILPVKPDIDTAVVGVSQCDLIMMAQNPGGKERSEEEFRALATEAGFKGVNLICCVCNFWVMEFCK

SEQ ID NO: 12 - protein, 506 aa, Nicotiana
MDLLLLEKTLIGLFFAIIVAIVVSKLRSKNFKLPPGPIPVPVFGNWLQVGDDLNHRNLTEYAKKFGDMFLLRMGQRNLVVVSSPELAKEVLHTQGVEFGSRTRNVVFDIFTGKGQDMVFTVYGEHWRKMRRIMTVPFFTNKVVQQYRRGWEDEVAHVVEDVKKNPESATNGIVLRKRLQLMMYNNMYRIMFDRRFESEDDPLFNKLKALNGERSRLAQSFEYNYGDFIPILRPFLRGYLNICKEIKQRRLQLFKDYFVDERKKLANTTKSMDNNSLKCAIDHILEAEQKGEINEDNVLYIVENINVAAIETTLWSIEWGIAELVNHPEIQKKLRDEIDSVLGVGVQITEPELNKLPYLQAVIKETLRLRMAIPLLVPHMNLHDAKLAGYDIPAESKILVNAWWLANNPATWKKPEEFRPERFFEEEKHVEANGNDFRYLPFGVGRRSCPGIILALPILGITLGRLVQNFELLPPPGQSKLDTTEKGGQFSLHILKHSTIVMKPRSF

SEQ ID NO: 13 - protein, 298 aa, Nicotiana
MGRKPCCVKEGLRKGPWSSKEDLLLTNYIKENGEGQWRSLPKNAGLLRCGKSCRLRWMNYLRPGIKRGNFSQDEEDLIVRLHSLLGNRWSLIAGRLPGRTDNEIKNYWNTHLIKKLKNAGIEPKPHKNFSKCSKKESRKGPQQGKSRKIQGKKSNNKNNKGQIVQVEKTKVFFPKPIRISCGISRNNSFENVTLSTTCSSNSNSGEANLENKENEVKLEEVSFFPRDLDFGKLLEGDAIYDEFLMEESCHISNKCSLPMNESMLEKVYEEYLLLLSENCYLQDDHQNEQNFPVNVSDQ

SEQ ID NO: 14 - protein, 381 aa, Nicotiana
MASEAHAAVHAPPPVAPTVCVTGAAGFIGSWLVMRLLERGYNVHATVRDPENKKKVKHLFELPKADTNLTLWKADLSVEGSFDEAIQGCQGVFHVATPMDFESEDPENEVIKPTVRGMLSIIESCAKANTVKRLVFTSSAGTLDAQEHQKLFYDETSWSDLDFIYAKKMTGWMYFVSKILAEKAAMEAAKKKNFDFISIIPPLVVGPFLTPTFPPSLITALSLITGNEAHYCIIKQGQYVHLDDLCEAHIFLYEQPKAEGRFICASHHAIIYDVAKMVREKWPEYYVPTEFKGIDKDLPVVYFSPKKLTDMGFQFKYTLEDMYKGAIETCRQKQLLPFSTQSTADNGRDKETIPLSAENYASGKENSPVANGTGKSTNGEI

SEQ ID NO: 15 - protein, 382 aa, Nicotiana
MASEGHAAVHAPSPPAAPTVCVTGAAGFIGSWLVMRLLERGYNVHATVRDPENKKKVKHLLELPKADTNLTLWKADLSVEGSFDEAIQGCQGVFHVATPMDFESEDPENEVIKPTVRGMLSIIESCAKANTVKRLVFTSSAGTVDVQEHQKLLYDETSWSDLDFIYAKKMTGWMYFVSKILAEKAAMEAAKKKNIDFISIIPPLVVGPFLAPTFPPSLITALSLITGNEAHYSIIKQGKYVHLDDLCEAHIFLYEHPKAEGRFICASHHAIIYDVAKMVQEKWPEYYVPTEFKGIDKDLSVVYFSSKKLTDMGFQFKYTLEDMYKGAIETCRQKQLLPFSTRSTADNVRDKEAIPLSTENYASGKENSPVANGTGKSTNGEI

SEQ ID NO: 16 - protein, 213 aa, Nicotiana
MGRKPCCSKEGLRKGTWTAKEDMLLTNYINEHGEVGWRSLPMKAGSRWSLIAGRIPGRTDNEIKNYWNTHLLKKLKSEGLEPKIHKSLAKNTRRQKEKANVSSQINQKGYKEKKKRNKKGNIEENCNNIEEKEQVAKKIEEQWHTQDSVQAMSGFSSTSEVASEKETNCNNVHCPSSGQSLEENDNEIYEKLQASGDSKRCKLNFSAEVNKTP

SEQ ID NO: 17 - protein, 435 aa, Nicotiana
MKIEVKESTMVKPAAETPQQRLWNSNVDLVVPNFHTPSVYFYRPTGSPNFFDGKVLKEALSKALVPFYPMAGRLCRDEDGRIEIDCKGQGVLFVEAESDGVVDDFGDFAPTLELRQLIPAVDYSQGIQSYALLVLQITHFKCGGVSLGVGMQHHAADGASGLHFINTWSDMARGLDLTIPPFIDRTLLRARDPPQPQFPHVEYQPPPTLKVTPENTPISEAVPETSVSIFKLTRDQINTLKAKSKEDGNTVNYSSYEMLAGHVWRSTCMARGLAHDQETKLYIATDGRSRLRPSLPPGYFGNVIFTTTPIAVAGDIQSKPIWYAASKLHDALARMDNDYLRSALDYLELQPDLKALVRGAHTFKCPNLGITSWSRLPIHDADFGWGRPIFMGPGGIAYEGLSFILPSPTNDGSQSVAISLQAEHMKLFEKFLYDF

SEQ ID NO: 18 - protein, 436 aa, Nicotiana
MGSEKMMKINIKESTLVKPSKPTPTKRLWSSNLDLIVGRIHLLTVYFYKPNGSSNFFDSKIMKEALSNVLVSFYPMAGRLARDEQGRIEINCNGEGVLFVEAESDAFVDDFGDFTPSLELRKLIPTVDTSGDISTFPLIIFQVTRFKCGGVSLGGGVFHTLSDGLSSIHFINTWSDIARGLSVAIPPFIDRTLLRARDPPTSSFEHVEYHPPPSLISSSKSLESTSPKPSTTTMLKFSSDQLGLLKSKSKHDGSTYEILAAHIWRCTCKARALSDDQLTKLHVATDGRSRLCPPLPPGYLGNVVFTGTPMAKSSELLQEPLTNSAKRIHSALSKMDDNYLRSALDYLELLPDLSALIRGPTYFASPNLNINSWTRLPVHDSDFGWGRPIHMGPACILYEGTVYILPSPNSKDRNLRLAVCLDADHMPLFEKYLYEF

SEQ ID NO: 19 - protein, 715 aa, Nicotiana
MASNGHVNGGENFELCKKSADPLNWEMAAESLRGSHLDEVKKMVSEFRKPMVKLGGESLTVAQVAAIAVRDKSANGVKVELSEEARAGVKASSDWVMDSMNKGTDSYGVTTGFGATSHRRTKNGGALQKELIRFLNAGVFGNGTETSHTLPHSATRAAMLVRINTLLQGYSGIRFEILEAITKLINSNITPCLPLRGTITASGDLVPLSYIAGLLTGRPNSKAVGPNGETLNAEEAFRVAGVNGGFFELQPKEGLALVNGTAVGSGMASMVLFDSNILAVMSEVLSAIFAEVMNGKPEFTDHLTHKLKHHPGQIEAAAIMEHILDGSSYVKAAQKLHEMDPLQKPKQDRYALRTSPQWLGPQIEVIRAATKMIEREINSVNDNPLIDVSRNKALHGGNFQGTPIGVSMDNARLALASIGKLMFAQFSELVNDYYNNGLPSNLTASRNPSLDYGFKGAEIAMASYCSELQFLANPVTNHVQSAEQHNQDVNSLGLISARKTAEAVDILKLMSSTYLVALCQAIDLRHLEENLKNAVKNTVSQVAKRTLTMGANGELHPARFCEKELLRIVDREYLFAYADDPCSCNYPLMQKLRQVLVDHAMNNGESEKNVNSSIFQKIGAFEDELKAVLPKEVESARAALESGNPAIPNRITECRSYPLYRFVRKELGTELLTGEKVRSPGEECDKVFTAMCNGQIIDPMLECLKSWNGAPLPIC

SEQ ID NO: 20 - protein, 341 aa, Nicotiana
MDNSAPDSLSRSETAVTYDSPYPLYAMAFSSLRSSSGHRIAVGSFLEDYNNRIDILSFDSDSMTVKPLPNLSFEHPYPPTKLMFSPPSLRRPSSGDLLASSGDFLRLWEINEDSSTVEPISVLNNSKTSEFCAPLTSFDWNDVEPKRLGTCSIDTTCTIWDIEKSVVETQLIAHDKEVHDIAWGEARVFASVSADGSVRIFDLRDKEHSTIIYESPQPDTPLLRLAWNKQDLRYMATILMDSNKVVILDIRSPTMPVAELERHQASVNAIAWAPQSCKHICSGGDDTQALIWELPTVAGPNGIDPMSVYSAGSEINQLQWSSSQPDWIGIAFANKMQLLRV

SEQ ID NO: 21 - protein, 440 aa, Nicotiana
MSMSVALLWVVSPTSEVSNGTGLLDSVREGNRVFVSSRFLARDRNLMWNGRIKKGGRQRWNFGSLIADPRYSCLGGSRTEKGSSFSVQSSLVASPAGEMTVSSEKKVYDVVLKQAALVKRQLRSTDELEVKPDIVVPGNLGLLSEAYDRCGEVCAEYAKTFYLGTKLMTPERRRAIWSIYVWCRRTDELVDGPNASHITPQALDRWEARLEDIFSGRPFDMLDAALSDTVSRFPVDIQPFRDMIEGMRMDLWKSRYNNFDELYLYCYYVAGTVGLMSVPVMGIAPESKATTESVYNAALALGLANQLTNILRDVGEDARRGRVYLPQDELAQAGLSDEDIFAGRVTDKWRNFMKKQIQRARKFFDESEKGVTELDSASRWPVSTALLLYRKILDEIEANDYNNFTRRAYVSKPKKLLTLPIAYAKSLVPPNRTSSPLAKT

SEQ ID NO: 22 - protein, 440 aa, Nicotiana
MSMSVALLWVVSPTSEVSNGTGLLDSVREGNRVFVSSRFLARDRNLMWNGRIKKGGRQRWNFGSLIADPRYSCLGGSRTEKGSSFSVQSSLVASPAGEMTVSSEKKVYDVVLKQAALVKRQLRSTDELEVKPDIVVPGNLGLLSEAYDRCGEVCAEYAKTFYLGTKLMTPERRRAIWAIYVWCRRTDELVDGPNASHITPQALDRWEARLEDIFSGRPFDMLDAALSDTVSRFPVDIQPFRDMIEGMRMDLWKSRYNNFDELYLYCYYVAGTVGLMSVPVMGIAPESKATTESVYNAALALGLANQLTNILRDVGEDARRGRVYLPQDELAQAGLSDEDIFAGRVTDKWRNFMKKQIQRARKFFDESEKGVTELDSASRWPVLAALLLYRKILDEIEANDYNNFTRRAYVSKPKKLLTLPIAYAKSLVPPNRTSSPLAKT

SEQ ID NO: 23 - protein, 248 aa, Nicotiana
MEGSSKGLRKGAWTTEEDSLLRQCINKYGEGKWHQVPVRAGLNRCRKSCRLRWLNYLKPSIKRGKLSSDEVDLLLRLHRLLGNRWSLIAGRLPGRTANDVKNYWNTHLSKKHEPCCKIKMKKRDITPIPTTPALKNNVYKPRPRSFTVNNDCNHLNAPPKVDVNPPCLGLNINNVCDNSIIYNKDKKKDQLVNNLIDGDNMWLEKFLEESQEVDILVPEATTTEKGDTLAFDVDQLWSLFDGETVKFD

SEQ ID NO: 24 - DNA, 992 bp, Nicotiana
atggaaagcaagagttccggaggcggagaaggaaaggttgtatgtgtaacaggggcctctggtttcatagcttcatggcttgttaagatgctacttcaacgtggttacactgtcaatgccactgttcgcaacctcaaggatgcgagtaaagtggatcacctgttaggccttgacggagctaaagagaggctgcatcttttcaaagctgagttacttggtgagcattcgtttgatcctgccgttgatggttgtgaaggtgtctttcatacagcatcacctgtttctctcacagctaaatccaaggaggaacttgtagaccctgctgtgagcggaacattaaacgtccttaggtcatgtaccaaatcaacatctgttagaagagtggtcataacctcttctaccgcttctgttatttgcaataaaaacatgtcaacccctggagctgtagctgatgagacttggtattcagatgcagaactctgtgaggaaagaaaggaatggtatcaactctccaaaaccttggctgaggaagctgcttggaaatttgcaaaggagaatgggttggacttggttacacttcatccaggtctagtcatcggtccacttctgcagcctacgctcaatttctcgtgcgaggctatagtgaacttcataaaagaaggaaaagaagcatggtctggcggaatatatagatttgtcgatgttagggatgttgctaatgcacatatactagcatttgaggtcccttcagcaaatggaagatattgtttagttggggtaaatggatattcttctttggttttgaagattgtacaaaagctttacccttccatcactctccctgagaattttgaagatggattacctcttatcccaaccttccaagtatcaagcgaaagagcaaaaagtttaggcgtcaatttcacatctcttgagttgagcgtgaaggacactgttgaaagcttgatagagaagaacttcctcaagatttg

SEQ ID NO: 25 - DNA, 1251 bp, Nicotiana
atgatgtgcaatattatttcacttgtgtccatcatcaacttctttttgctgttttatagagttgttgtcctaccacaacatgctgctgcttctcactctaccgttgaatttcttcctggatttgaaggtccacttcctttccatcttgagactgggtatattggagtaggtgaatatgaagaagtgcagctcttttattattttcttaaatcagaatcagaacccacaaaagatcctattttgatttggctctcaggaggacctggttgctcttcctttactgcacttgtttatcaaatagggcccttgtattttgagccaaacgagtataatgggagccttccaaagctaacattgaatccaaactcatggaccaaggtagctaacataatattcttggatcaacctgtgaatagtggcttctcttatgcaacaacttcaacaacattcaagtctactgatctacaagcatgccaccatatctaccagtttttgcgaaagtggttgattaagcatcaagagttcattaggaatccaatgtacattggtggagattcatattctggcatcactgttccagttatcactcaactaatatcaaatggaattgaagcagggcacaagccatcgattaatcttaagggatatatacttgggaatcctagcacgtttcctcttcaatataactactgggttccttatgctcatggaatgggacttatctccgacgaactttatcaggctactactcttatcctttactttaaaatttatcatatcataaatgcaattaatttagcttacatggttgaggtacacaggttgtctacttactgggcaaatgatccaagagtacaagaagctcttaatgttcgtaagggagctataacaagatggacaagatgtagggaaagtatcgtgaataaaacttacactattactttccaagatagcataccttatcatgtggaactcagcaaaaaactttatcgatcacttatatacagtggcgatcatgatatgggcattccattccaatcaactcaattttggataaaatctctaaattattctattgtggatgaatggcggccatggagttttgatggtcaagttgcaggatatacaagatcctattccaaccagatgacatttgcaactgtcaagggagcaggacatgtagctcctgagtacaagcctaaagagtgctttaccatgtttcaaagatggttgtctcatgaaccactttga

SEQ ID NO: 26 - DNA, 1710 bp, Nicotiana
atgttgagtgtagctagtgttgaagcccagaaagcagagttatcttcttctgtaattcctccttctgatcaatctactgaagagatacacgtgtttagatcaagattaccagatatacaaatttccaacaatgttcctcttcatgtttacttgtttgagaggctctctgaatttcaagataggacatgtcttatagcaggcagcagtggacaatcctacacttttgctgaaactcatctcatttgccagaaaatagctgctggcttaacaaatataggaatcaaaaagggagatgtaatcatgacttttctccagaactgcgcggaatttgtgtttacttttctctcggcttctatgattggcgccgttataactacagctaatccattttacacaaaagcagaggcgtttaagcaattaaaagcgtcgaatgcaaaactaatcgttactcaatctcagtacgtggataaatttcgtgattctggagagaatgacccgaaaattggcgaagatttttcagtcattacaattgatgacccccctgaaaattgcttacatttctctgtactttctgaagctaacgaagaggaaatgccaaagggaattgtaatccaaccagatgatccagtagctttaccattttcttcaggaacaacagggctaccaaaaggtgtgattttaactcacaaaagtttaatcacaggagtagctcaattagtcgacggagataatccaaatttgtacttaaaacaagacgacgtggtgctatgtgtgctacctttgtttcacatatttgcgttaaattcagtgcttttagtctcgttaagagcaggagctagtgttttactaatgcaaaaattcgaaattggtgcattgctggagctgatacaaaaccaccgcgtgtcagttgcagcagtagttccgcccttggttcttgcgttggcgaaaaatccgatggttgattcgttcgatttgagttcgattaggctcgtgttgtccggggcggcgccgctggggaaagagttggaggaagcgctacatcaaagagtcccgcaagctatatttggtcaggggtatggtatgacagaggcaggaccagtagtaacaatgtgcccagcatttgcaaagcaaccattttcaaccaaatctggctcatgtggttcagtagttcgaaatgcagacctcaaggtggtcgaccccgaaactggtggctccctcggccgcaaccaacccggcgaaatttgcatccgtggttcccaaatcatgaaaggttatctgaatgatgatgaggccacggcacggaccatagatgtcgatggatggctccacactggtgatataggatacgtagatgacgatgatgaaatatacatcgtcgatagagtcaaagagcttatcaagttcaaaggattccaggtgccaccagctgagcttgagtcccttctagtaagccatccagatattgcagatgctgctgttgtaccgcaaaaagatgatgcggcaggggaagtcccagttgcatttgtggtccgctccgccaatggttttgaaattactgaagaagctataaaggaatttattgccaaacaggtgatattctataaaagattgcacaaggtgtattttattcacgctattccaaagtctccgtctggaaagatactgaggaaagaactgagagccaaactagctgcgccctccacccagtga

SEQ ID NO: 27 - DNA, 1656 bp, Nicotiana
atgggaactcgtgcagtagaaagctcacagcagcaagaatgtgaacatattttccggagtagatatcctccggttcaagtaccggacaatgtgaccctcccggattttgtgcttcacaatgtagagttatacactgacaaaatggcatttgtggatgctaccactggcaaaggctacacttatggccaagttgcaagagacataaggaggttcgccaaggccttgagatcccttggcttaaggaaaggacgggtggtggtggtagttcttccaaatgtaccagaatatgctattgttgctcttggaatcatggctgctggtggcgtcttctccggtgcaaatccagcagctcattcatcagaaatcgtgaaacaagttgaatctgctgatggcaagcttattgtctctgatctaccaacctatcacaaggttaaagattgtgggctgccagtaataatactaggtgaagaacatgtagaaggaacaattcattgggatgaattgcttgaagctgcagagcgtgccggttccagaactgatcacataacaaaccatgaagatgaaatggtgcagcaaaatgatttatgtgcactgcccttctcgtcaggcactacggggctgtccaagggagtgatgttaacccacagaaatctagtagcaaacctctgctctacactcttcagtgttagcccagaaatggtaggccaagttacaacactgggtttgataccattcttccacatttatgggataactggaatctgttgtgcaaccattagaaacaaagggaaagtggtagtcttgcgtaggtacgaactgagggcatttctaaatgcactcattacacatgaagtcacatttgcaccaattgtgccacctatcatcttggcacttgttaagaatcctattgtggatgaatttgatctcagcaagcttaagcttagatccatcatgacagcggcagccccacttgcccctgagattcttaatgaatttgaaaagaaatttcccgatgttcaggtccaagaggcatatgggatgactgagcacagctgcattactctttctcatagtgaccagcatactgctaaaagaaattctgttggttttattctacctaatttggaggtaaagttcgttgatcctgataccggtagatctctccccaaaaacaaaccaggcgagatatgtgtcaaaagccaatgtgttatgaagggttactacaaaaatgaatttgagacttgccttaccattgataaggatggatggcttcagactggtgacattggctacattgacgatgatggagatatcttcctagtcgatcgtatcaaagagcttatcaagtacaagggattccaagttgctccagctgagttagaagggatccttctcacacatccttcagtagaagatgctgcagtagttgggctgccagatgaagaagcaggagagataccagtggcatgggtagtcttgaactcaaaagcaaaagaaagcgaagaggacattatcaactacattgcatcgactgttgcacagtataaacgagtgagagtggtgcagttcgttgatagtattccaaaatctccttctggaaaaatactgagaagacttatcaaggataagatgctagagagacttaagaatgcatag

SEQ ID NO: 28 - DNA, 2016 bp, Nicotiana
atgacggagataccgcctaacagccagatgaaaaccatgttgcagaaggcagtgcaatcggttcaatggacatatactcttttctggcaattatgtccccaacaaggggcgttagtgtggagagatggatattacaatggggctataaagactagaaagacagtgcagccaatggaagttagcgctgaggaagcttctcttcacagaagccaacagcttagagaactttacgaatcactttccgccggcgagtcaaatcagccagcgagaaggccgtcggcagctttgtcaccggaggacttgacggagtccgagtggttttatctcatgtgtgtttctttctcttttcctcctggcatcggattacctggcaaggcttattcgaagaaacatcacatatggatcatgggcgcaaacgaggttgatagcaaagtcttctgtagagctattcttgccaagagcgcccgcatacagacggtcgttggtattcctctcttggatggtgtactggaactgggaactacagaaagggttcaagaagagattggattcataaaccatgtaaagagctttttcactgagcaacaacaacctcagctaccaaagccagccttatctgagcactccacttccaatcccaccaccttttccgagccacatttttactccggcaatacttcgccatctgctaatgttgatattgcgcatcaagatggcggagctgccggcgaagaagatgaggaggaggaagaagaagaagatgatgatgaagccgagttggactcggatagtatagcgattcaaagcgcggctaatcctattgccgttgaggctagtgaactcatgcagcttgatgtgtccgaggctatacagctcggctcgcccgatgatgactctgataatatggactctgattttcatttggttggcgctggaaacacggctcatgactaccagcgccaagctgactctttcaaagccgagaccgccattagctggccgcacttccaagaccttcaacaattaccaggtggctctagttatgatgaattatcacaagaagacacacactattctcaaacagtgtcaaccattctcgaacaccgaagctccaaattttcctctacaacaatgggctgtatttctcatgactcggcccaatctgccttcacattgtgccctagcaccaccgtctgcagcccgaatcccgcccactgccgccacgacgactcacttgtcgacggtggcggcgcctcccagtggctgctcaaaagcatactcttcactgtcccatttcttcacactaaataccaatctgaagcttctccaaagtcacgtgacgtcgccactgttgattcctccagtactgcttctcgctttcgcaaaggctgtagtataacgtcgcaagaagagccaagtggaaaccatgtacttgcagaacgacgtcgtagagagaagctaaatgagcgttttatcatattaaggtctcttgtaccttttgtaacgaaaatggacaaagcctccattttgggtgacaccatagagtatgtcaagcagttacgtaagaaagttcaggatcttgaagctcgtgctcgcgacacggagcactccagagatgcagataaaaaaggtggcacagctacagtgaaggtgttgcaaggaaggggtaagaggagaatgaatacggtagatggaagtgttggtggagggcaggcaacgataacggcgtccccaccgtcaacgacggaaaatgaggaggttgtgcaagtacaagtatcaattatcgaaagcgatgcattggtggagctccggtgtccgtacaaagaggggttgctgttaaatgtaatgcagatgctaagggaactcaaagtggaagttgtagccattcaatcagctcttaataatggcgtcttcttggctgagttaagagctaaggtaaaagagaatatatgtggaaggaaagcaagcattttggaagtaaaaaggtcaatacatcagataatccctagagattaa

SEQ ID NO: 29 - DNA, 2052 bp, Nicotiana
atgacggagataccgcctaacagccagatgcaaaccatgttgcagaaggctgtgcaatcggttcaatggacatatactcttttctggcaattatgttcccaacaaggggtgttagtgtggagagatggatattacaatggggctataaagactagaaagactgtgcagccaatggaagttagcgctgaggaagcttctcttcacagaagccaacagcttagagaactttacgaatcactttccgccggcgagtcaaatcagccggcgagaaggccgtcggcagctttgtcaccggaggacttgacggaatccgagtggttttatctcatgtgtgtttctttctcttttcctcctggcatcggattacctggcaaggcttattcaaagaaacatcacatatggattatgtgcgcaaacgaggttgatagcaaagtcttctgtagagctattcttgccaagagtgcccgcatacagacggtcgtctgtattcctctcttggatggtgtactggaactgggaactacagaaagggttcaagaagacattggattcataaaccatgtaaagagctttttcactgagcaacaacaacctcagccaccaaagccagccttatctgagcactccacttccaattccaccaccttttccgagccacacttttactccggcaatactccgccatctggcaatgctgatattgcgcagcaagatggcggagctgccggagaagaagatgaggaggaggaagaagaagaagacgatgaagccgagttggattcggatagtatagcaattcaaagtgaggttggtggcgcggctaatcctatagcggctgaggctagtgaactcatgcagcttgatatgtctgaggctatacggcttggctcgcccgatgatggctctaataatatggactctgattttcatttggttggcgctggaaatacggctgactaccagcgtcaacctgactctttcaaagccgagactgccattagctgggctcacttccaagaccttcaacatttaccaggtggctctagttatgaagaattatcacaagaagacacacattattctcaaacagtgtcaaccattcttgaacacttctcaaaccgaagctccaaattttcctctaccacaatgggctgtatttctcatgactcagcccaatctgccttcacattgtgccctagcaccaccgtcgactgcagcccgaatcccgcccactgccgccgccgccacgacgattcacttctcgacggtggcggcgcctccccctcctcccagtggctgctcaaaagcatactcttcactgtcccatttcttcacactaaataccaatctgaagcttctccgaaatcagttgacgtcgccactgttgattcctccagtactgcttctcgctttcgcaaaggctgtagtataacgtcgcaagaagagcccagtggaaaccatgtacttgcagaacgacgtcgtagagaaaagctaaatgagcgttttatcatattaaggtctcttgtaccttttgttacgaaaatggataaagcctccattttgggtgacaccatagagtatgtcaagcagttacataagaaagttcaggatcttgaagctcgtgctcgtcacacggagcagtccaaagatgcagaccaaaaaagtggcacagctacagtgaaggtgttgcaagggaggggtaagaggagaatgaatacggtggaggccggaaatattggtggagggcaggcaaagatgacggcttttccgctatcaacaacggaggatgaagaggttgtgcaagtagaagtatcaattattgaaagcgatgcattgttggagctccgatgtccgtacaaagaggggctgctgttagatgtaatgcagatgctaagggaactcaaggtggaagttgtagccattcaatcatctcttaataatggcatcttcttggctgagttaagagctaaggtaaaagagaatatatatggaaggaaagcaagcattgtggaagtaaaaaagtcaatacatcagataatccctagagattaa

SEQ ID NO: 30 - DNA, 663 bp, Nicotiana
atgaatatttgtactaataagtcgtcgtcaggagtgaagaaaggtgcatggactgaagaagaagatgttctattgaaaaaatgcatcgagaaatatggagaaggaaagtggcatcaagttcctcttagagctggtttgaatagatgcagaaagagctgcagattaaggtggctaaattatctaaggccacatataaagagaggagacttctcttttgatgaagtagatctcattttgaggcttcataagctgttaggcaacagatggtcacttattgctggtagacttcctggaaggacggcaaacgatgtcaaaaactactggaacagccatcttcgcaagaagttaattgctcctcatgatcaaaaggagagcaagcaaaaagcaaagaagatcaccatattcagacctcggcctcgaaccttctcaaagacaaatacttgtgttaaaagtaacacaaatactgtagataaggatattgaaggcagcagcgaaataattagattcaacgataatttgaagccaacaactgaagaattgacggatgatggaattcaatggtgggccgatttactagctaacaattacaacaataatgggattgaggaagctgataattcatcaccaactttgttgcatgaggaaatgccacttctcagttga

SEQ ID NO: 31 - DNA, 1260 bp, Nicotiana
atggtggtgatcagtgcagtagttccaactccttcaagagttgaaagcttggctaaaagtggaatccaggctatccctaaagagtatgtgaggccacaagaagagttaaatggaataggaaacatatttgaggaagagaagaaagatgaaggacctcaagtaccgacgattgatctgaaagaaatcgactcagaggacaaggaaattcgcgagaaatgccacaaagagttgaagaaagcagctatggagtggggtgttatgtaccttgttaaccatggcatatcagatcagctaattgatcgtgtcaaggttgctggaaagaccttctttgatcaacctgttgaagaaaaggagaagtatgctaatgaccaaccctctggcaatgtccaaggctatggcagcaagttagcaaatagtgcttgtggtcagcttgaatgggaggattatttcttccattgcgttttccccgaggacaagtgcgacttatccatctggcctaaaatccctactgactacattccagcaacaagtgaatatgccaaacagattaggaacctagcaacaaagattttggcagtgctttctattgggctgggactagaagaaggaagactagagaaggaagtcggaggcaaggaggacctactgcttcaaatgaagattaactactaccccaaatgtccccaaccagaactagcacttggcgttgaagctcatactgatgtgagtgcactgacttttatcctccacaatatggtgcctgggttacaacttttctatgaaggacagtgggtaacggcaaagtgtgtgcctaattccataatcatgcatattggggacacccttgaaatcctaagcaatggaaagtacaaaagcattcttcacagaggggttgtgaataaagagaaagtaagaatctcatgggctattttctgtgagccgccaaaggagaagatcatccttaagcccctatctgagactatcactgaggctgaaccacctcgattcccacctcgcacctttgcacagcatatggcccataagctcttcaagaaggatgatcaggatgctgctgctgaacacaaagtctccaagaaggatgacccggattctgctgctggacacaaacccttcaagaaggatgatcaggatgctgttgttcagcaaaaagtcctcaaggaggatgaacaggatgccgctgctgagcacaaagtcttcaagaaggataatcaggatgctgctgctgaagaatctaaatag

SEQ ID NO: 32 - DNA, 1260 bp, Nicotiana
atggtggtgatcagtgcagtagttccaactccttcaagagttgaaagcttggctaaaagtggaatccaggctatccctaaagagtatgtgaggccacaagaagagttaaatggaataggaaacatatttgaggaagagaagaaagatgaaggacctcaagtaccgacgattgatctaacagaaatcgactcagaggacaaggaaattcgagagaaatgccaccaagagttgaagaaagcagctatagaatggggtgttatgcaccttgttaaccatggcatatcagatgagctaattgatcgtgtcaaggtttctggagataccttctttgatcaacctgttgaagaaaaggagaagtatgctaatgaccaaccctctggcaatgtccaaggctatggcagcaagctagcaaatagtgcttgtggtcagcttgagtgggaggattatttcttccattgtgttttccctgaggacaagtgcaacttatccatctggccgaaaacccctacagactacattccagcaacaagtgaatatgccaagcagatcaggaacctagcaacaaagattttggcagtgctttctattgggctgagactagaagaaggaagactagagaaggaagtcggaggcatggaggacctgctgcttcaaatgaagattaactactatcccaaatgcccccaaccagaactagcacttggtgtcgaagctcatactgatgtcagtgcactgacttttatcctccacaatatggtgcctggcttgcaacttttctacgaaggacagtgggtaacggcaaagtgtgtgcctaattccataatcatgcatattggggacacccttgaaattctaagcaatggaaagtacaagagcattcttcacagaggggttgtgaataaagagaaaataagaatctcatgggctattttctgtgagccgccgaaggagaagatcatccttaagcccctacctgagactataactgaggctgagccacctcgattcccacctcgcacctttgcacagcatatggcccataagctcttcaagaaggatgatcaggatgctgctgctgaacacaaagtctccaagaaggatgacccggattctgctgctgaacacaaacccttcaagaaggatgatcaggatgctgttgctcagcaaaaagtcctcaaggaggatgaacagaatgccgctgctgagcacaaagtcttcaagaaggataatcaggatgctgctgctgaagaatctaaatag

SEQ ID NO: 33 - DNA, 1869 bp, Nicotiana
atggctatgggacaccaagaccaagatggagttccaaacaacttgagaaagcaacttgctcttgctgttagaggtattcaatggagctatgcaatcttctggtcaactccagttacacagccaggggtgttggaatggagtgatgggtactataatggggatatcaagactaggaagacagttcaggtgggggaagttaatgaagaccaacttgggttgcacagaactgagcaattgcgagaactttatagttcactcttaacaggtgaaggtgaagaagacttacaacctcaggctaaaaggccctcagctgcattatctcctgaagatctcactgatacggagtggtatttcttagtatgcatgtctttcgtcttcaatgttggacaagggttgccagggaagacctcagcgacgaatcaaacaatctggctatgcaatgctcaccaagcagagagtagagtattttctcgctctctgctagcaaagagtgcatctatccagactgtcgtatgctttccatatttaggaggcgttattgagctgggagtcaccgagcttgtcttagaagatcccaacctcattcagcaaataaaaaattcctttgaggttgatcactctgttatttcgaagaggcctaattacaactccaatgatgcaaaagatgacatgaatgttgctagccgaaagcttgatcataatgtacttgaaagtgatgcttatccagttgaaataaacaacagttcaccgcatgatagttcaaacggttttgtggccaatcaagaggcagaagattctttaatggtggtaggcgttataggggaaacttcacaagctcaaagctggaagttcgtggatgataatatgagtaacggtgtgcataattctttgaattccagtgactgcatctctcaaaattatgaaaagttgtcccctctttcgaatggagaaaaagaaactaagccttgcccaatagaccgtcaagagcacaatcagaataaactgcatcttttagatcaccaaggagatgacgctcaatatcaagctgtcatttctacccttttaaaaagctctgaccaattaactttgggaccacattttagaaatattaacaaaaagtcaagctttgctggttggaagaatgatactgaagcgccaagaataggaactgcacaaaaactattgaagaaggtacttcttgaagttcctagaatgcatggtggtgttacacataaattcagcagagagaatcgtaaaaagaacggcctttggagaccggaggttgatgacattgatagaagccgtgttatttcagagagaaggcgaagagaaaagataaacgagagatttatgcatcttgcatcaatgctgccgactggtggcaaggttgacaaaatatcactacttgacgagacaatagaatacatgaaagagcttgagaggagagttcaagagctggaagctagatcaggaaaaaaaacaaatgatactgcagagcagacatctgataattgtggcactagtaaattcaatgacgtcaatggatcgttaaagaggaaagcatgtgatatggatgaaatggaacctgaaagctgtaatgaattactgaaaggcagttcagctgatggtattgtcatcagtatgatcgataaggaagtctcgatcaagatgaggtgtctttggagcgagggcttgttacttaagattatggaggcactaaccgacctacaaatggattgccatacggttcaatcttccaagattgatgggattttatccattgctattgaatcaaagtcaaatggattgaaaactgtatcagttggagcaattagagaagtacttcagcgagtagtctggaaatcttga

SEQ ID NO: 34 - DNA, 1095 bp, Nicotiana
atggaatcctcaaccaaaagccaaataccaacacaatcagaagaagagcgtaactgcacatatgccatgcaactattgtcatcttcagtcctcccctttgtgttgcattcaacaattcaattggaagtttttgagatattagccaaatctaatgacactaaactttctgcttctcaaattgtttctcaaattcctaactgcacaaaacctgaagcacctactatgttaaataggatgctttatgtcttggctagttactccttgtttacttgttccattgttgaagatgaaaaaaataatgggggccaaaaaagagtgtatggtttgtcacaagtgggaaaattctttgttaaaaatgaaaatggtgcatcaatggggccacttttggctttgcttcaaaataaagtattcataaacagctggtttgaactaaaagatgcagttcttgaaggaggagttccatttgacagggtacacggtgtgcatgcatttgaatatccaaaatcggacccaaaattcaatgatgttttcaacaaggcaatgatcaatcacacaactgtagtcatgaaaaaaatacttgaaaattacaaaggttttgagaaccttaaaactttggttgatgttggaggtggtcttggagttaacctcaagatgattacatctaaataccccacaattaagggcactaattttgatttgccacatgttgttcaacatgccccttcctatcctggggtggaacatgttgggggagatatgtttgaaagtgttccagaaggagatgctatttttatgaagtggattcttcatgactggagtgatagtcacaacctcaagttgctaaagaactgctacaaggctctaccagacaatggaaaggtgattgttgttgaggccattttaccagtgaaaccagacattgacaccgcagtggttggcgtttcgcaatgtgatttgatcatgatggctcaaaatcctggaggcaaagagcgatcggaagaggagtttcgagccttggctactgaagctggattcaaaggcgttaacttaatatgttgtgtctgtaatttttgggtcatggaattctgcaagtag

SEQ ID NO: 35 - DNA, 1521 bp, Nicotiana
atggatcttctccttctagagaagacccttatagggttattctttgctatcattgtagctatagttgtttctaagctacgtagcaagaattttaagttgcccccaggtccgattcctgtgccagtttttggcaattggcttcaagttggtgatgacttgaatcacagaaacctcactgaatatgccaagaaatttggtgacatgttcttgctaagaatgggacagaggaatcttgtggtggtgtcatcccctgaactagccaaagaagttttgcatacacaaggggttgaatttggatcaagaacaaggaatgtggtctttgatattttcactggaaaaggccaagatatggtttttacagtatatggtgaacactggaggaaaatgaggaggattatgactgttccattttttacaaacaaagtggtgcagcagtataggcgtgggtgggaagatgaagtggcacatgttgttgaggatgtgaagaaaaatccagagtcagcaactaatgggattgtgttgaggaaaaggttgcagcttatgatgtacaataacatgtacaggattatgtttgataggaggtttgagagtgaggatgatcctttgtttaacaagcttaaggctttgaatggggagaggagtagattggctcagagttttgagtacaattatggtgattttatccctatattgagacctttcttgagaggttacttgaacatctgtaaggaaattaagcagaggaggttgcagcttttcaaagattactttgttgatgaaagaaagaaacttgcaaacacgacgaagagcatggacaataattcgctaaagtgtgccattgatcacattcttgaggctgaacagaagggagagatcaatgaggataatgtcctttacattgttgagaacatcaatgttgctgcaatagaaactacactgtggtcaatcgagtggggtattgctgaactagtgaaccaccctgaaatccagaagaaactccgtgacgagattgacagtgttcttggagtaggagtgcaaatcactgagccagaactcaacaagcttccttaccttcaggctgtgatcaaggagacccttcgtctccgtatggcaatccctcttttagtcccacacatgaaccttcacgatgcgaagcttgctggatatgacattcccgcggagagcaagatcctggtaaacgcttggtggctggctaacaaccctgctacctggaagaagcccgaagagtttaggccagagaggttctttgaagaggagaagcacgttgaggctaatggcaatgacttcagatatcttccatttggtgttggtaggaggagctgccctggaattatccttgcactgccaattcttggcattaccttgggacgcttggtgcagaactttgagttgttgcctcctccaggacagtcaaagcttgacacaacagagaaaggcgggcaattcagtctgcacattttgaagcattccaccattgtgatgaaaccaagatctttttaa

SEQ ID NO: 36 - DNA, 897 bp, Nicotiana
atgggaagaaaaccatgttgtgtaaaagagggattgagaaaaggtccatggtcttctaaagaagatttattacttactaattatatcaaggaaaatggtgaaggacaatggagatctttgcctaagaatgctgggttgcttaggtgtggaaaaagttgtagactaagatggatgaactatttaagaccagggattaaaagaggaaatttcagtcaagatgaagaagatcttatagtgagactacattctcttttgggtaatcgttggtcactaattgctggaagattaccaggtcgtacagacaatgaaatcaagaattattggaacacacatttaatcaagaagctcaaaaatgctggaattgaaccaaaaccccacaaaaatttctccaaatgttccaaaaaggaatcaagaaaaggaccccaacaagggaaatcaagaaaaatacaaggcaaaaagagcaacaacaaaaacaataagggtcaaattgtacaagttgagaagaccaaagtatttttcccaaaacccatcaggatttcttgtggaatttcaaggaacaatagttttgaaaatgttacattgagtactacttgttcctcaaatagtaattctggagaagctaatcttgaaaacaaggaaaatgaggtgaaattagaagaagtttcattctttccaagggacttagattttggtaaattacttgaaggggatgcaatttatgatgaatttctaatggaagaaagttgccacatttcaaacaaatgttcattgccaatgaatgagagcatgttggagaaagtatatgaagaatatcttttacttctttctgaaaattgttaccttcaagatgatcatcaaaatgagcaaaatttccctgtaaatgtttctgatcagtga

SEQ ID NO: 37 - DNA, 1146 bp, Nicotiana
atggcaagtgaagctcatgcagctgttcatgctcctcctccggtagcaccgacggtttgcgtcactggagcagctggatttattggctcttggcttgtcatgagactccttgaacgtggttataatgttcacgctactgttcgtgatcctgagaacaagaagaaggtaaagcatctattcgaattgccaaaagctgacacaaacttaacgctgtggaaagcggacttgtcagtggaaggaagctttgatgaagccattcaaggctgtcaaggagtattccatgtggcaacacctatggatttcgagtccgaggaccctgagaatgaagtaattaaaccaacagtcaggggaatgttaagcatcatagaatcatgtgctaaagcaaacacagtgaagaggctggttttcacttcatcggctggaactctcgatgcccaagaacaccaaaagcttttctatgacgagaccagctggagcgacttggacttcatatatgctaagaagatgacaggatggatgtattttgtttccaagatactggcagagaaggccgcaatggaagcagctaaaaagaagaactttgattttattagcatcataccgccgctggttgttggtccattcctcacgcctacattcccacctagcttaatcactgcactttcactaattactgggaatgaagctcactactgcatcattaaacaaggtcaatatgtgcatttggatgatctttgtgaggctcatattttcctatatgagcagccaaaggcagagggaagattcatctgcgcgtcccatcatgctatcatctatgatgtggcaaagatggtccgagagaaatggccagagtactacgtccctactgagtttaaaggcatcgataaggacttgcccgtggtgtatttttcgccaaagaagctgacggatatggggtttcaattcaagtacactttggaggatatgtataaaggggccattgagacttgtcgacagaagcagttgcttcccttttctacccaaagcacagcagataatggacgtgacaaagaaaccattcccctttctgctgaaaactatgcaagtggcaaagagaattcaccagttgcaaatggtacaggaaagtcaaccaatggggaaatctag

SEQ ID NO: 38 - DNA, 1149 bp, Nicotiana
atggcaagtgaaggtcatgcagctgttcatgccccttctcctccggcagcgccgacagtttgcgtcactggagcagctggatttattggctcttggcttgtcatgagactccttgaacgtggttataatgttcacgctactgttcgtgatcctgagaacaagaagaaggtaaagcatctattggaattgccaaaagctgacacgaacttaacgttgtggaaagcagacttgtcagtggaaggaagctttgatgaagccattcaaggctgtcaaggagtattccatgtggcaacgcctatggatttcgagtccgaggatcctgagaatgaagtaattaaaccaacagtcaggggaatgttaagcatcatagaatcatgtgctaaagcaaacacagtgaagaggctggttttcacttcatctgctggaactgtcgatgtccaagagcaccaaaagctcttatatgacgagaccagctggagtgacttggactttatatatgctaagaagatgacaggatggatgtattttgtttccaagatactggcagagaaggccgcaatggaagcagctaaaaagaagaacatcgatttcattagcatcataccgccactggttgttggtccattcctcgcgcctacattcccacctagcttaatcactgccctttcactaattactgggaatgaagctcactacagcatcattaaacaaggtaaatatgtgcatttggatgatctttgtgaggctcatattttcctatatgagcacccaaaggcagaggggagattcatctgcgcgtcccatcatgctatcatctatgatgtggcaaagatggtccaagagaaatggccggagtactacgtccctactgagtttaaaggcatcgataaggacttgtccgtggtgtatttttcgtcaaagaagctgacggatatggggtttcaattcaagtacactttggaggatatgtataaaggggccattgagacttgtcgacagaagcagttgcttcccttttctacccgaagcactgcagataatgtacgtgacaaagaagccattcctctttctactgaaaactatgcaagtggcaaagaaaattcaccagttgcaaatggtacgggaaagtcaaccaatggtgaaatctag

SEQ ID NO: 39 - DNA, 642 bp, Nicotiana
atgggaagaaaaccctgttgttctaaagaaggtctgaggaaaggtacatggactgcaaaagaagatatgctacttactaattatattaatgaacatggagaagttggatggagatctcttcctatgaaagctggaagtcgttggtctctcattgctggaagaatacctggtcgaacagacaacgaaataaagaattattggaacacacatcttctcaagaaactcaaatccgaaggacttgagccaaaaatacacaaatctcttgcaaaaaacactagaagacaaaaggagaaagcaaatgtttcttcccaaattaaccaaaaaggttacaaggaaaagaagaagaggaataaaaagggcaatatcgaagaaaattgtaacaatattgaagagaaagaacaagtagctaagaagatagaggagcagtggcatacgcaggattccgtgcaagcgatgtcagggttttcaagtactagtgaagttgctagtgagaaggaaactaattgcaataatgtccattgtccttcttctggtcaaagtcttgaagaaaatgacaatgaaatttatgagaagcttcaggctagcggagattctaaacgttgcaaattgaatttcagtgcagaggttaataagaccccttaa

SEQ ID NO: 40 - DNA, 1308 bp, Nicotiana
atgaagatcgaggtgaaagaatcgacgatggtaaagccggcggcggagacgccacaacagaggctgtggaactctaatgtggatttggtggtgccgaatttccacacgccaagtgtttatttttacaggccgacgggatccccaaatttcttcgacggaaaagtgctgaaggaagctctaagcaaagcacttgtgccgttttatcctatggcggggaggctgtgtagggacgaagatggtcgtattgagattgactgtaaaggtcagggggtgctttttgtggaagctgagtcggatggtgtggtggatgattttggtgattttgccccgacgttagaactccgtcaactcatccccgccgttgattactcacaaggaattcaatcgtatgctctcttagtgttgcagataacacattttaaatgtgggggagtttcccttggtgtgggcatgcaacatcatgcagcagatggagcttctggtcttcacttcatcaacacatggtctgatatggctcgtggtctggacctcaccatcccacctttcattgaccggaccctcctccgtgctcgtgatccacctcagcctcagtttccccatgtcgagtaccagccacctcccactctcaaggtaactccagaaaacacccctatatctgaagctgttcctgaaaccagcgtgtccatcttcaaattaacccgtgatcaaatcaataccctcaaagcgaagtccaaggaagatggaaataccgttaactacagctcctacgagatgttggcaggacatgtgtggcgctccacgtgcatggcacgaggactcgctcatgatcaagaaaccaaattgtacatagcaacagatggacgttccaggcttcggccctctctcccaccaggctatttcggtaatgtgatatttactaccactcctattgcagtcgcaggtgatatccaatcgaagcctatttggtatgctgccagtaaattacatgatgcattggctagaatggacaacgattacttaagatcagctcttgattatttggagttgcagcctgacttaaaggctcttgttcgtggtgcacatacgtttaagtgcccgaatttaggaataactagttggtctaggctgccaatccatgatgctgattttggctggggtaggcctatatttatgggacctggtggtattgcttatgaaggtttaagctttatattgccaagtcctacaaatgatggcagtcaatctgttgcaatctctctacaagcagaacacatgaaacttttcgagaagttcttgtatgacttttga

SEQ ID NO: 41 - DNA, 1311 bp, Nicotiana
atgggaagtgaaaaaatgatgaaaattaatatcaaggaatcaacattagtaaaaccatcaaaaccaacaccaacaaaaagactttggagttctaacttagatttaatagtgggaagaattcatcttttaacagtatatttctataaaccaaatggatcttcaaatttctttgattcaaaaataatgaaagaagcattaagtaatgttcttgtttcattttacccaatggctggaagattagctagagatgaacaaggaagaattgagataaattgtaatggagaaggagttttatttgttgaagctgaaagtgatgcttttgttgatgattttggtgattttactccaagtttggaacttaggaaacttattcctactgttgacacttctggtgatatttctactttccccctcatcatctttcaggttactcgtttcaaatgtggtggagtttcacttggtggaggagtattccacactttatcagatggtctctcatcaattcacttcatcaacacatggtccgatatagcccgaggcctctccgtcgccatcccgccgttcatcgaccggaccctcctccgtgcacgggacccaccaacatcgtctttcgagcacgtcgagtatcatcctcctccatctctaatttcatcatcaaaaagcttagaatccactagcccaaagcctagtaccacaaccatgttaaaattctctagtgaccaacttgggcttctaaagtccaagtccaaacatgatggtagcacttacgaaatcctcgcggcccatatttggcgttgcacgtgcaaggcacgtgcactgtccgacgatcaattgaccaaattacatgtggccactgatggtaggtctaggctttgccctcctttgccaccaggttacttaggaaatgttgtgttcacaggcacacctatggcaaaatcaagtgaacttttacaagaaccattgacaaattcagccaagagaattcatagtgcattatcaaaaatggatgacaattacctaagatcagctctcgattacctcgaattactgcccgatttatcggctttaatccgtggaccgacgtactttgctagccctaatcttaatattaatagttggactagattgcctgttcatgattcagattttggatggggaaggccaattcatatgggaccagcttgcattttatatgaagggacagtttatatattgccaagtccaaatagtaaagataggaacttgcgtttggctgtttgtttagatgctgatcacatgccactatttgagaagtatttgtatgaattttga

SEQ ID NO: 42 - DNA, 2148 bp, Nicotiana
atggcatcaaatggtcatgttaatggaggagaaaactttgagttgtgcaaaaaatcagctgatccattgaattgggaaatggcagctgaatccttaagagggagtcatttggatgaagtgaaaaaaatggtgagtgaatttagaaaaccaatggtaaaacttggtggtgaaagtttaacagtggcacaagtggctgctattgctgttagggacaaaagtgcaaatggtgttaaagttgaactttctgaagaggcaagagctggtgttaaagctagtagtgattgggttatggacagtatgaataaaggaactgatagttatggtgttactactggttttggtgctacatctcataggagaaccaagaatggtggtgctcttcaaaaagaacttattaggttcttgaatgctggtgtttttggcaatggaacagaaacaagccacacattgccacattcagcaacaagggcagctatgcttgttaggatcaacacactcctacaaggctactctggcatcagatttgaaatcttggaagctattacaaaattgattaacagcaacatcactccatgtttacctctccgtggaacgatcactgcctcgggtgatcttgtccctttatcctacattgctggtttgctcactggtaggcctaattccaaggctgttggtcccaatggtgagacacttaatgctgaagaagcgttccgcgttgctggtgttaacggtggatttttcgagttgcagcctaaggaaggacttgcacttgtgaatggtacagctgttggttctggtatggcatcaatggtcctctttgattccaacattcttgctgtaatgtctgaagttttatcagcaattttcgctgaagtaatgaacggaaagcccgaattcactgaccatttgacacacaagttgaagcaccaccctggtcaaattgaggctgctgctattatggaacatattttggatggaagctcttatgtgaaggcggctcaaaagctacatgaaatggatcctctacaaaaaccaaagcaagatcgttatgctctccgaacatctccacaatggcttggccctcaaattgaagtcattcgcgctgcaactaagatgattgagagggagattaactcagtgaacgataaccctttgatcgatgtttcaagaaacaaggcgttacatggtggcaacttccaaggcactcctatcggtgtttccatggataatgcaagattggctcttgcatcaattgggaaattgatgtttgctcaattctcggaacttgtcaacgactattacaacaacggtttgccctctaatctcactgcatcaaggaatccaagcttggactatggtttcaagggagctgaaatcgccatggcttcttactgctcagaacttcaattcttggcaaatccagtgacaaaccatgtccaaagtgctgaacaacacaaccaagatgtcaactccttaggcttaatctcagcaaggaaaacagctgaagctgttgatatcttaaagctcatgtcatcaacttatctcgtggcactttgccaagctatagacttgaggcatttggaagaaaacttaaagaatgcagtcaagaacacagttagccaagtagctaagagaactcttacaatgggtgctaatggtgaacttcatccagcaagattctgtgaaaaggaattgcttcgaatcgtggatagggaatacttgttcgcctacgctgatgatccttgcagttgcaactaccctttaatgcagaaactgagacaagtacttgttgatcatgcaatgaataatggtgaaagtgagaagaatgtgaacagctcaatctttcaaaagattggagctttcgaagatgaattgaaggctgttttaccaaaggaagttgagagtgcaagagctgcattagaaagtggaaaccctgctattcctaacaggattacagaatgcagatcttatccattgtacaggtttgtgagaaaggagcttggaacagaattattgacaggagaaaaagtccgatcaccgggcgaggagtgtgacaaagtgttcacagcaatgtgcaatggacaaatcattgatccaatgttggagtgtctcaagagctggaatggtgctcctcttcctatctgttag

SEQ ID NO: 43 - DNA, 1026 bp, Nicotiana
atggataattcagctccagattcgttatccagatcggaaaccgccgtcacatacgactcaccatatccactctacgccatggctttctcttctctccgctcatcctccggtcacagaatcgccgtcggaagcttcctcgaagattacaacaaccgcatcgacattctctctttcgattccgattcaatgaccgttaagcctctcccgaatctctccttcgagcatccttatcctccaacaaagctaatgttcagtcctccttctctccgtcgtccttcctccggagatctcctcgcttcctccggcgatttcctccgtctttgggaaattaacgaagattcatcaaccgtcgagccaatctcggttctcaacaacagcaaaacgagcgagttttgtgcgccgttgacttccttcgattggaacgatgtagagccgaaacgtctcggaacttgtagtattgatacgacgtgtacgatttgggatattgagaagtctgttgttgagactcagcttatagctcatgataaagaggttcatgacattgcttggggagaagctagggttttcgcatcagtctctgctgatggatccgttaggatctttgatttacgtgataaggaacattctacaatcatttacgagagtcctcagcctgatacgcctttgttaagacttgcttggaacaaacaagatcttagatatatggctacgattttgatggattctaataaggttgtgattctcgatattcgttcgccgactatgcctgttgctgagcttgaaagacatcaggctagtgtgaatgctatagcttgggcgcctcagagctgtaaacatatttgttctggtggtgatgatacacaggctcttatttgggagcttcctactgttgctggacccaatgggattgatccgatgtcggtttattcggctggttcggagattaatcagttgcagtggtcttcttcgcagcctgattggattggtattgcttttgctaacaaaatgcagctccttagagtttga

SEQ ID NO: 44 - DNA, 1323 bp, Nicotiana
atgagcatgtctgttgctttgttgtgggttgtttctcccacttccgaggtctcgaatgggacaggattgttggattcagtccgagaaggaaaccgcgtctttgtatcatccaggttcctagctcgagataggaatttgatgtggaatgggagaatcaagaaaggtgggagacaaaggtggaattttggctctttaattgctgatccaagatattcatgcttgggtggatcaagaactgaaaagggaagcagtttctctgtacagtccagtttggtggctagcccagctggagaaatgacagtgtcatcagagaaaaaggtctatgatgtggtattgaagcaagcagctttagtgaagaggcagctgagatctaccgatgaattagaagtgaaacctgatatagttgttccagggaatttgggcttgttgagtgaagcatatgatcgttgtggcgaagtatgtgcagagtatgcaaagacattttacttaggaacaaagctaatgactccagagagaagaagagctatctggtcaatatatgtgtggtgcaggagaacggatgagctagtcgatggccctaacgcatcacacataactccacaagctttagacaggtgggaggccaggctggaagatattttcagtgggcggccatttgatatgcttgatgctgctttatccgatactgtctccagatttcctgttgatattcagccattcagagatatgatagaaggaatgcgtatggacttgtggaaatccagatataacaacttcgatgagctatatctctattgttattatgttgctggtacagtaggactgatgagtgttccagttatgggtattgcacctgaatcaaaggcaacaacagagagtgtatataatgctgctttggctttagggcttgcaaatcaactaaccaatatactcagagatgtaggagaagatgccagaagaggacgagtatacttacctcaagatgaattagcacaggcagggctttctgatgaagatatatttgctggaagagtgaccgataagtggaggaactttatgaagaaacaaattcagagggcgaggaaattctttgatgagtcagagaaaggtgtcacagaactggactctgctagtagatggcctgtaagtacagcgctgctgttgtatcgcaagatattggacgagattgaagccaatgactacaataacttcacaaggagggcttatgttagcaagccaaagaagcttctcaccttgcccattgcttatgcaaaatctcttgtgccccctaatagaacttcctctccactagcaaaaacatga

SEQ ID NO: 45 - DNA, 1323 bp, Nicotiana
atgagcatgtctgttgctttgttgtgggttgtttctcccacttccgaggtctcgaatgggacaggattgttggattcagtccgagaaggaaaccgcgtctttgtatcatccaggttcctagctcgagataggaatttgatgtggaatgggagaatcaagaaaggtgggagacaaaggtggaattttggctctttaattgctgatccaagatattcatgcttgggtggatcaagaactgaaaagggaagcagtttctctgtacagtccagtttggtggctagcccagctggagaaatgacagtgtcatcagagaaaaaggtctatgatgtggtattgaagcaagcagctttagtgaagaggcagctgagatctaccgatgaattagaagtgaaacctgatattgttgttccagggaatttgggcttgttgagtgaagcatatgatcgttgtggcgaagtatgtgcagagtatgcaaagacattttacttaggaacaaagctaatgactccagagagaagaagagctatctgggcaatatatgtgtggtgcaggagaacggatgagctagtcgatggccctaacgcatcacacataactccacaagctttagacaggtgggaggccaggctggaagatattttcagtgggcggccatttgatatgcttgatgctgctttatccgatactgtctccagatttcctgttgatattcagccattcagagatatgatagaaggaatgcgtatggacttgtggaaatccagatataacaacttcgatgagctatatctctattgttattatgttgctggtacagtaggactgatgagtgttccagttatgggtattgcacctgaatcaaaggcaacaacagagagtgtatataatgctgctttggctttagggcttgcaaatcaactaaccaatatactcagagatgtaggagaagatgccagaagaggacgagtatacttacctcaagatgaattagcacaggcagggctttctgatgaagatatatttgctggaagagtgaccgataagtggaggaactttatgaagaaacaaattcagagggcgaggaaattctttgatgagtcagagaaaggtgtcacagaactggactctgctagtagatggcctgtgttagcagcgctgctgttgtatcgcaagatattggacgagattgaagccaatgactacaataacttcacaaggagggcttatgttagcaagccaaagaagcttctcaccttgcccattgcttatgcaaaatctcttgtgccccctaatagaacttcctctccactagcaaaaacatga

SEQ ID NO: 46 - DNA, 747 bp, Nicotiana
atggagggttcgtccaaagggctgcgaaaaggtgcttggactactgaagaagatagtctcttgagacagtgcattaataagtatggagaaggcaaatggcaccaagttcctgtaagagctgggctaaaccggtgcaggaaaagttgtagattaagatggttgaactatttgaagccaagtatcaagagaggaaaacttagctctgatgaagtcgatcttcttcttcgccttcataggcttctagggaataggtggtctttaattgctggaagattacctggtcggaccgcaaatgacgtcaagaattactggaacactcatctgagtaagaaacatgaaccgtgttgtaagataaagatgaaaaagagagacattacgcccattcctacaacaccggcactaaaaaacaatgtttataagcctcgacctcgatccttcacagttaacaacgactgcaaccatctcaatgccccaccaaaagttgacgttaatcctccatgccttggacttaacatcaataatgtttgtgacaatagtatcatatacaacaaagataagaagaaagaccaactagtgaataatttgattgatggagataatatgtggttagagaaattcctagaggaaagccaagaggtagatattttggttcctgaagcgacgacaacagaaaagggggacaccttggcttttgacgttgatcaactttggagtcttttcgatggagagactgtgaaatttgattag

SEQ ID NO: 47 - protein, 717 aa, Nicotiana
MASNGHVNGGENFELCKKSSATDPLNWEMAAESLRGSHLDEVKKMVSEFRKPMVKLGGETLTVAQVAAIAVRDKSANGVKVELSEEARAGVKASSDWVMDSMNKGTDSYGVTTGFGATSHRRTKNGGALQKELIRFLNAGVFGNGTETSHTLPHSATRAAMLVRINTLLQGYSGIRFEILEAIAKLINSNITPCLPLRGTITASGDLVPLSYIAGLLTGRPNSKAVSPNGETLNAEEAFRVAGVNGGFFELQPKEGLALVNGTAVGSGMASMVLFDSNILAVMSEVLSAIFAEVMNGKPEFTDHLTHKLKHHPGQIEAAAIMEHILDGSSYVKAAQKLHEMDPLQKPKQDRYALRTSPQWLGPQIEVIRAATKMIEREINSVNDNPLIDVSRNKALHGGNFQGTPIGVSMDNARLALASIGKLMFAQFSELVNDYYNNGLPSNLTASRNPSLDYGFKGAEIAMASYCSELQFLANPVTNHVQSAEQHNQDVNSLGLISARKTAEAVDILKLMSSTYLVALCQAIDLRHLEENLKNAVKNTVSQVAKRTLTMGANGELHPARFCEKELLRVVDREYLFAYADDPCSCNYPLMQKLRQVLVDHAMNNGESEKNVNSSIFQKIGAFEDELKAVLPKEVESARAALECGNPAIANRITECRSYPLYRFVRKELGTELLTGERVRSPGEECEKVFTAMCNGQIIDPMLECLKSWNGAPLPIC

SEQ ID NO: 48 - protein, 712 aa, Nicotiana
MAGVAQNGHQEMDFCMKVDPLNWEMAADSLKGSHLDEVKKMVAEFRKPVVKLGGETLTVAQVAAIAAKDNVKTVKVELSEGARAGVKASSDWVMDSMGKGTDSYGVTTGFGATSHRRTKNGGALQKELIRFLNAGVFGNGTESCHTLPQSGTRAAMLVRINTLLQGYSGIRFEILEAITKLLNHNVTPCLPLRGTITASGDLVPLSYIAGLLTGRPNSKAVGPNGETLNAEEAFRVAGVNGGFFELQPKEGLALVNGTAVGSGLASMVLFDANVLAVFSEVLSAIFAEVMNGKPEFTDHLTHKLKHHPGQIEAAAIMEHILDGSSYVKAAQKLHETDPLQKPKQDRYALRTSPQWLGPQIEVIRSATKMIEREINSVNDNPLIDVSRNKALHGGNFQGTPIGVSMDNARLALASIGKLMFAQFSELVNDYYNNGLPSNLTAGRNPSLDYGFKGSEIAMASYCSELQFLANPVTNHVQSAEQHNQDVNSLGLISARKTAEAVDILKLMSSTYLVALCQAIDLRHLEENLRNAVKNTVSQVAKRTLTMGTNGELHPSRFCEKDLLRVVDREYVFAYADDACSANYPLMQKLRQVLVDHALQNGENEKNANSSIFQKILAFEDELKAVLPKEVESARAALESGNPAIANRIKECRSYPLYRFVRGELGAELLTGEKVRSPGEECDKVFTAMCNGQIIDSLLECLKEWNGAPLPIC

SEQ ID NO: 49 - protein, 389 aa, Nicotiana
MVTVEEFRRAQRAEGPATVMAIGTATPSNCVDQSTYPDYYFRITNSEHKTELKEKFKRMCEKSMIKKRYMHLTEEILKENPNICAYMAPSLDARQDIVVVEVPKLGKEAAQKAIKEWGQPKSKISHLVFCTTSGVDMPGCDYQLTKLLGLRPSVKRFMMYQQGCFAGGTVLRMAKDLAENNKGARVLVVCSEITAVTFRGPNDTHLDSLVGQALFGDGAAAVIVGSDPIPDVERPLFELVSAAQTLLPDSEGAIDGHLREVGLTFHLLKDVPGLISKNIEKSLVEAFQPLGISDWNSLFWIAHPGGPAILDQVELKLGLKQEKLKATRNVLSNYGNMSSACVLFILDEMRKASAKEGLGTTGEGLEWGVLFGFGPGLTVETVVLHSVAT

SEQ ID NO: 50 - protein, 369 aa, Nicotiana
MAPSTLTALAEEKTLQTSFIRDEDERPKVAYNQFSDEIPIISLKGIDDEGGINGRRGEICEKIVKACEDWGVFQVVDHGVDAQLISQMTTLAKQFFALPAEEKLRFDMSGGKKGGFIVSSHLQGEVVQDWREIVTYFSYPIRARDYSRWPDKPEGWIDVTQKYSEKLMELACKLLEVLSEAMGLEKEALTKACVDMDQKVVVNFYPKCPQPDLTLGLKRHTDPGTITLLLQDQVGGLQATKDNGKTWITVQPVVGAFVVNLGDHGHFLSNGRFKNADHQAVVNSNSSRLSIATFQNPAPEAIVYPLKIREGEKAVMDEPVAFAEMYRRKMSKDLELARLKKLAKEQQIQAEEAAEKAKSETKPIDEILA

SEQ ID NO: 51 - protein, 145 aa, Nicotiana
MFGPQSGKDGWTDLTFMYDMIRIRDKSLCSSFLQIFSSEGCKMLEMTCEEHDKLAARSQFLTHTIGRILSEMEVEPTPIDTKGFQKLVQVKESSVRDSFDLFSGLFIHNRFARQQMKNLEVAVEKTKQKLEERSKELQDPIISKF

SEQ ID NO: 52 - protein, 376 aa, Nicotiana
MLSFTPLQSKPTPPTPTSNPTRWSWSHLTHHHPTTRRHFSASSPSKVSYRRLSINAIDAAQPYDYEALVSNQYAQSTRLKIAIVGFGNFGQFLAKAFVRQGHVVFAHSRTDYSHIANSLGVLFFQDPHDLCEQHPDVILLCTSIISTEPVLRSLPIQRLKRNTLFVDVLSVKEFPKNIFLQVLPSHFDILCTHPMFGPESGKDSWKDLAFVFDKVRIGEGESRKGRVDRFLDIFEKEGCRMVQMTCAEHDRYAAGSQFITHTMGRVLEKLDLETTPINTKGYETLLNLVENTSSDSFDLYYGLFMYNKNAMEQLERLDLAFEALKKELFGHLHEVLRKQLFGKAEEAGQRRILTKLPKNGYALPAPSSEAVKSENN

SEQ ID NO: 53 - DNA, 2154 bp, Nicotiana
atggcatcaaatggtcatgttaatggaggagaaaactttgagttgtgcaagaaatcatcagccactgatccattgaattgggaaatggcagctgaatctttaagagggagtcatttggatgaagtgaaaaaaatggtgagtgaatttagaaaaccaatggtaaaacttggtggtgaaactttaacagtggcacaagtggctgctattgctgttagggacaaaagtgcaaatggtgttaaagttgaactttctgaagaggcaagagctggtgttaaagctagtagtgattgggttatggatagtatgaataaaggaacagatagttatggtgttactactggttttggtgctacatctcataggagaaccaagaatggtggtgctcttcaaaaagaacttattaggttcttgaatgctggtgtttttggcaatggaacagaaacaagccacacattgccacattcagcaacaagggcagctatgcttgttaggatcaacacactcctacaaggctactctggcatcagatttgaaatcttggaagcaattgcaaaattgattaacagcaacattactccatgtttacctctccgtggcacgatcactgcctcgggcgatcttgttcctttatcctacattgctggtttgctcactggtaggcctaattccaaggctgttagtcccaatggtgagacccttaatgctgaagaagcgttccgcgttgctggtgttaacggtggatttttcgagttgcagcctaaggaaggacttgcacttgtgaatggtacagcagttggttctggtatggcatcaatggtcctctttgattccaacattcttgctgttatgtctgaagttttatcagcaattttcgctgaagttatgaacggaaagcccgaatttactgaccatttgacacacaagttgaagcaccaccctggtcaaattgaggctgctgctattatggaacatattttggatggaagctcttatgtgaaggcggctcaaaagctacatgaaatggatcctctccaaaaaccaaagcaagatcgttatgctctccgaacatctccacaatggcttggccctcaaattgaagtcattcgcgctgcaactaagatgattgagagggagattaactcagtgaacgataaccccttgatcgatgtttcaagaaacaaggcattacatggtggcaacttccaaggcacccctatcggtgtgtccatggataatgcaagattggctcttgcatcaattgggaaattgatgtttgctcaattctcggaacttgtcaacgactattacaacaacggtttgccatctaacctcaccgcatcaaggaatccaagcttggactatggtttcaagggagctgaaatcgccatggcatcttactgctcagaacttcaattcttggcaaatccagtgacaaaccatgtccaaagtgctgagcaacacaaccaagatgtcaactccttgggcttaatctcagcaaggaaaacagctgaagctgtcgatatcttaaagctcatgtcatcaacttatctagtggcactttgccaagctatcgacttgaggcatttggaggaaaacttaaagaatgcagtcaagaacacagttagccaagtagctaagagaactcttacaatgggtgctaacggtgaacttcatccagcaagattctgtgaaaaggaattgctacgagtcgtggacagggaatacttgttcgcctacgctgatgatccttgcagttgcaactaccctttaatgcagaaactgagacaagtacttgttgatcatgcaatgaataatggtgaaagtgagaagaatgtgaacagctcaatcttccaaaagattggagctttcgaagacgaattaaaggctgttttaccaaaggaagttgagagtgcaagagctgcattggaatgtggcaaccctgctattgctaacaggattacagaatgcagatcttatccattgtacaggtttgtgagaaaggagcttggaacagaactactaacaggagaaagagtccgatcaccgggcgaggagtgtgagaaagtgttcacagcaatgtgcaatggacagattattgatccaatgttggagtgtctcaagagctggaatggtgctcctctacctatctgttag

SEQ ID NO: 54 - DNA, 2139 bp, Nicotiana
atggctggtgttgcacaaaatggtcaccaagaaatggatttttgcatgaaagtggatccattaaactgggaaatggcagctgattcattgaaaggaagccatttagatgaagtgaagaaaatggtggctgagtttaggaaaccagtagtgaaacttggaggtgagactttgacagtggctcaagttgcggctattgctgcaaaagataatgttaaaactgttaaagtggagctttctgaaggggcaagagctggtgttaaagctagcagtgattgggttatggacagtatgggtaaaggaactgatagttatggtgttacaactggctttggtgctacttcacataggaggaccaagaatggtggtgctcttcaaaaggaacttattaggttcttgaatgctggagtttttggcaatggaacagagtcatgtcacacattaccacaatcagggacaagggcagctatgttagttaggatcaacactctccttcaagggtactctggcatcagatttgaaatcttagaagcaatcactaaattgcttaaccacaatgttactccatgtttgccccttcgcggcaccatcaccgcctctggtgatctcgtccccttgtcctacattgccggtttactcactggtcggcctaattctaaagcagttggacctaatggcgaaaccctcaacgctgaagaagcgtttcgtgttgctggagttaacggtggatttttcgagttgcagcctaaggaaggccttgctcttgtgaatggtactgcagttggttctggtttggcctcaatggttctctttgatgctaatgttctcgcggtcttttctgaagttctctcagctatttttgctgaggtaatgaatggaaagcccgagttcactgaccacttgacacacaagttgaagcatcaccccggacaaattgaggctgctgctattatggaacacattttggatggtagctcttatgtgaaggcggctcagaagcttcacgaaacggatcctctccaaaaaccaaagcaagatcgttatgctcttagaacgtcgccccaatggcttggccctcaaattgaggtcatccgttctgcaaccaagatgattgagagggagattaattcagtgaacgacaaccctttgatcgatgtttcaagaaacaaggcattacacggtggcaacttccagggcactccaattggtgtctctatggacaatgctagattagcccttgcatcaatagggaaattgatgtttgcccaattctccgagcttgtcaacgattactacaacaacggattgccatctaatctgacagcaggaaggaatcctagcttggactatggtttcaagggatctgagattgccatggcttcatactgttcagaacttcaattcttggcaaatccagtgactaaccacgtacaaagcgccgagcaacacaaccaagatgtgaactccttgggcttaatctcagctagaaaaacagctgaagccgtggacatcttaaagctaatgtcatccacatatctagttgcactttgccaagcaatagacttgaggcatttggaagaaaatctgaggaatgcagtcaagaacacggtgagccaagtcgcaaagagaactttaacaatgggtaccaatggagaacttcatccatcaagattctgtgaaaaggacttgcttcgagtcgtggacagggaatacgtcttcgcctatgctgacgacgcctgcagcgctaactacccactgatgcagaaactaaggcaagtcctcgtcgaccacgccttgcaaaatggcgaaaatgagaagaacgcaaacagctcaatcttccaaaagatactagcttttgaagacgagctaaaggccgtgttgccaaaagaagtcgagagtgcaagagccgcgctggaaagtgggaaccctgcaattgccaacaggataaaagaatgcagatcttatccactttacaggtttgttagaggagaacttggagctgaattattgacgggagaaaaagtcaggtcaccaggtgaagaatgtgacaaagtgttcacagcaatgtgcaatggacaaattattgattcattgttagaatgtctcaaggaatggaatggtgcacctcttccaatctgttag

SEQ ID NO: 55 - DNA, 1170 bp, Nicotiana
atggtgacggtcgaggagtttcgtagggcacaacgtgccgagggtccggccacggtcatggccatcggaacagccacaccttccaactgtgttgatcaaagcacttaccccgattactattttcgtatcactaatagcgagcataagactgagcttaaggagaaatttaagcgcatgtgtgaaaaatcaatgattaagaaaaggtacatgcacttaacagaggaaatcttgaaagagaatcctaatatttgtgcatacatggcaccttcccttgatgctagacaagacatagtggtggttgaagtgccaaaacttggcaaagaggcagcccaaaaggccatcaaagaatggggccagcccaagtccaaaattagtcatttggtcttttgtacaactagtggtgtagacatgcccgggtgtgactaccaactcactaagctactcgggctccgtccttcggtcaagcggttcatgatgtaccaacaaggttgctttgccggtgggacggtactccggatggctaaggacttggccgaaaacaacaagggcgctcgagtccttgttgtttgctcagagatcaccgctgtcacgttccgtgggcccaatgacacccacttggatagtttggttgggcaagccctttttggtgatggggcagccgcggtcattgtaggttctgatccaattccagatgtcgagaggcctttgttcgagcttgtttccgcagcccaaaccctactccccgatagcgaaggcgctatcgacggtcatctccgtgaagttgggcttacattccacttactcaaagatgttcctgggcttatctcgaaaaacattgagaaaagccttgtggaagcattccaacctttgggaatttctgattggaactctttattttggattgctcaccctggtgggcctgccattttggaccaagttgaactaaaattgggcctaaagcaagagaaacttaaggctacaagaaatgtattaagtaactatggcaatatgtcaagtgcttgtgtgttgtttattttggatgaaatgaggaaagcctctgcaaaagaaggtttaggaactactggtgaagggcttgaatggggtgtgctttttggatttgggcctgggcttacagttgagactgttgtccttcacagtgttgctacttag

SEQ ID NO: 56 - DNA, 1110 bp, Nicotiana
atggcaccttcgacattgacagctctagcagaggaaaagacacttcaaacaagtttcataagagatgaagatgagcgaccaaaagtggcgtacaaccaattcagcgatgagattccgatcatatcgttgaagggtattgatgatgagggtggaattaatggaagaagaggtgaaatatgtgaaaagattgtcaaggcatgtgaagattggggcgttttccaggtagttgatcatggtgttgatgctcaacttatctcacaaatgacaactctcgctaaacaattcttcgctttgcctgctgaggaaaagctacggtttgacatgtcgggtggcaagaaaggtggcttcattgtctctagccatctacagggtgaagtggtccaagattggcgtgaaatagtgacctacttctcatacccaattcgggctagagactactctagatggccagacaaaccagagggatggatagatgtgactcaaaagtacagtgaaaagttaatggagttggcttgcaaattattggaagtactatcagaggctatgggcttagagaaggaggccttaaccaaggcatgtgtggatatggaccaaaaagtggttgtcaatttttacccaaagtgtccacagcctgaccttacccttgggctgaaacgacacactgatccaggaaccatcaccctcttgttacaagaccaagttggtgggcttcaagccactaaagataatggcaaaacttggattactgttcagcccgttgttggcgcttttgttgtcaatcttggtgaccatggtcattttttgagcaatggaaggtttaagaacgctgatcatcaagcagtggtgaactcgaatagcagcagattatcgatagctacgtttcagaatccagcaccagaggcaatagtgtatcctttgaaaattagggaaggagagaaggcagtgatggacgagcccgtagcatttgcagaaatgtataggaggaaaatgagtaaggaccttgagcttgctaggctcaagaaactagccaaggagcagcaaatacaagctgaagaagctgctgagaaggccaagtcggaaaccaagcctattgatgaaattcttgcttaa

SEQ ID NO: 57 - DNA, 438 bp, Nicotiana
atgtttggaccacaaagtggaaaagatggatggactgatttgacttttatgtacgacatgattcgaattagagataaatctctgtgttccagttttctgcaaatattctcaagtgaggggtgcaaaatgctggaaatgacttgtgaagagcatgacaaattggctgctcgaagtcaatttctgactcacacaattggcaggatcttatccgaaatggaggttgaacccacccccatagacacgaagggatttcagaaacttgttcaagtgaaggagagctcagttagagatagttttgatctattcagcgggctattcatacacaataggtttgccaggcaacagatgaaaaatttagaagtagcagtggagaaaactaaacagaagcttgaagagaggtcgaaggagctgcaggatcctatcatatctaagttctag

SEQ ID NO: 58 - DNA, 1131 bp, Nicotiana
atgttgtctttcacccctcttcaatccaagccaacaccacccacccccacctcaaaccccacccgttggtcttggtctcatctcacccaccaccaccccactacccgccgccacttctctgcctcttcaccctccaaagtcagttaccgccgccttagcattaatgccattgatgcagcacagccatatgattatgaagcattagtttcaaatcaatatgctcagtcaacaagactcaagattgctatagtgggttttggcaacttcggtcagtttcttgctaaagcctttgttcgtcaaggtcatgttgtttttgctcattcaagaactgattactcacacattgcaaattctttaggtgttttgttttttcaagatccacatgacctttgtgagcaacatcctgatgttattctactttgtacttcaattatatctactgaacctgtccttagatcactccctattcaaaggctaaaaagaaacacattatttgttgatgttttgtctgttaaagagtttccaaagaacattttccttcaagttttgccttcccattttgatattttgtgtactcatcctatgtttggacctgaaagtggtaaggatagttggaaagatttggcctttgtgtttgataaagttagaattggtgaaggggaatcgagaaaaggaagggttgataggtttcttgatatatttgagaaagaagggtgtaggatggtgcagatgacgtgtgcggagcatgataggtatgctgcaggttcgcagtttattacacatacaatggggagagtattggagaagttggatttggagacaactcctattaatacgaaagggtacgagactttgttgaatttggttgagaatacttctagtgatagctttgacttgtactatgggttgtttatgtacaataagaatgcgatggagcagttggaaagacttgatttggctttcgaggctttgaagaaggagttatttgggcatttgcatgaagtcttgaggaagcaattgttcgggaaggcggaggaagcgggacagagacgtatcttaaccaagttgcccaagaatgggtatgcactaccagctccttcatcggaggctgttaaatctgagaacaattga

SEQ ID NO: 59 - DNA, 2623 bp, Artificial Sequence
  comprises plant native sequences only
cccgggttagtattcaaaccgaataaatcaaagttaccaaaccgaataaatcgaaaccgaaaggagaaaccgcaccataccgaatttaattaggtacgatattgatattgtattttaaaaaatcgaataccaaaaataccgaattaaaatatctaaatatcgtacagtaccgaccgataaatactctataagcatcatcatgtcaccattcctgcttggaaatagatgtaataatgtaattcaaggtgaagatcattgaaaatgagatatttggactcttagataattgtgcaactgatatttttatttactttttttctttcatccaataattgcgttacattaaaaatgagatatttggattaatattcttctccttgaccacaaagcaaggaaagcctaaggaccgatagtaaagttgtattcgtgtggttgcgtgttagttttgagcggcaaaataaattatgttaaggtaaattatttttggaacaataataaaattatttctgtataatatataaatcatatatttgaaccgtagaattatcagttaatacttgtatatgaggaggctaactacgttagagcgctaacgagaatacttcatataccgtattttttacgataataataatgtaatgtgaaattgctatccaaaaggcacctaattttgtccaccgttcaaaggaaaggacaaggaagtagtagcgtgtaggtttggtgctgtacaaaataagcaagacacgtgttgccttattataggataatccataaggcaatttcgtcttaagtcggccattgcacctttaaaaggagcctctttgttcccaaaatcttcatcctttgatttctctattctcaatatctcctcaatttttctctagtcttcaaacacttctcaaggtacattaacttcttctttctttttgttcctcttattttatgctacttttatttaatttcgatctatatttttaggatctaaatactcatttttgatttgtttaatcgctctgtatatatgcaccaagttgaaatttttgtaagtttattttgttcggtctatattttaagatctgaaataccctttactgagaaaaaaaaaactcaaccttgattttgttgtacctggttgaatttgttattgttgtgtatacagttaaaaaactcaagtcttgattttattgtttcccttttgtagtttgtatatacatagagctgaattggtgttctaattttggttgatttttatgtatacagtataaaatcgatcttagttttgttcattgatttgtatttgcacaaagttggaattttgcgtttgttattttgatgattgaaaccttttctgtatatacagctcgagatggagggttcgtccaaagggctgcgaaaaggtgcttggactactgaagaagatagtctcttgagacagtgcattaataagtatggagaaggcaaatggcaccaagttcctgtaagagctgggctaaaccggtgcaggaaaagttgtagattaagatggttgaactatttgaagccaagtatcaagagaggaaaacttagctctgatgaagtcgatcttcttcttcgccttcataggcttctagggaataggtggtctttaattgctggaagattacctggtcggaccgcaaatgacgtcaagaattactggaacactcatctgagtaagaaacatgaaccgtgttgtaagataaagatgaaaaagagagacattacgcccattcctacaacaccggcactaaaaaacaatgtttataagcctcgacctcgatccttcacagttaacaacgactgcaaccatctcaatgccccaccaaaagttgacgttaatcctccatgccttggacttaacatcaataatgtttgtgacaatagtatcatatacaacaaagataagaagaaagaccaactagtgaataatttgattgatggagataatatgtggttagagaaattcctagaggaaagccaagaggtagatattttggttcctgaagcgacgacaacagaaaagggggacaccttggcttttgacgttgatcaactttggagtcttttcgatggagagactgtgaaatttgattagtctagaaataacagagggcgcgcgagcggtggctactgatcgcctatgagttctgtgattctacttgtaatttcagaagtgttttcagtgtcttgttttctggaagtccgtctggtttttagtaacttttagctcaaaaatgtgtctgtacgatggtatttgtatgtttgtgggtcttttacatatacgcttgtaatcgatcaatgtagaatgctgtgtgccttttccgtcaacagcttatttagtgtttactctgtatacgtatatctaatatatagtactgattctttcatctggtgatttgttttcctaaagagattattatcatagctttaattgaatgatacaaagaggtgttgcctggcttcaccagagcagaaattttcattgatatagggtacaaatgtcattcacataatgttaagagataagtttttcaatgtcctcaagagcccaccaagagtttcttccgggaattgcttaaattatcttaaatttaaattgtaaaac

SEQ ID NO: 60 - DNA, 2539 bp, Artificial Sequence
  plant native sequences only
cccgggttagtattcaaaccgaataaatcaaagttaccaaaccgaataaatcgaaaccgaaaggagaaaccgcaccataccgaatttaattaggtacgatattgatattgtattttaaaaaatcgaataccaaaaataccgaattaaaatatctaaatatcgtacagtaccgaccgataaatactctataagcatcatcatgtcaccattcctgcttggaaatagatgtaataatgtaattcaaggtgaagatcattgaaaatgagatatttggactcttagataattgtgcaactgatatttttatttactttttttctttcatccaataattgcgttacattaaaaatgagatatttggattaatattcttctccttgaccacaaagcaaggaaagcctaaggaccgatagtaaagttgtattcgtgtggttgcgtgttagttttgagcggcaaaataaattatgttaaggtaaattatttttggaacaataataaaattatttctgtataatatataaatcatatatttgaaccgtagaattatcagttaatacttgtatatgaggaggctaactacgttagagcgctaacgagaatacttcatataccgtattttttacgataataataatgtaatgtgaaattgctatccaaaaggcacctaattttgtccaccgttcaaaggaaaggacaaggaagtagtagcgtgtaggtttggtgctgtacaaaataagcaagacacgtgttgccttattataggataatccataaggcaatttcgtcttaagtcggccattgcacctttaaaaggagcctctttgttcccaaaatcttcatcctttgatttctctattctcaatatctcctcaatttttctctagtcttcaaacacttctcaaggtacattaacttcttctttctttttgttcctcttattttatgctacttttatttaatttcgatctatatttttaggatctaaatactcatttttgatttgtttaatcgctctgtatatatgcaccaagttgaaatttttgtaagtttattttgttcggtctatattttaagatctgaaataccctttactgagaaaaaaaaaactcaaccttgattttgttgtacctggttgaatttgttattgttgtgtatacagttaaaaaactcaagtcttgattttattgtttcccttttgtagtttgtatatacatagagctgaattggtgttctaattttggttgatttttatgtatacagtataaaatcgatcttagttttgttcattgatttgtatttgcacaaagttggaattttgcgtttgttattttgatgattgaaaccttttctgtatatacagctcgagatgaatatttgtactaataagtcgtcgtcaggagtgaagaaaggtgcatggactgaagaagaagatgttctattgaaaaaatgcatcgagaaatatggagaaggaaagtggcatcaagttcctcttagagctggtttgaatagatgcagaaagagctgcagattaaggtggctaaattatctaaggccacatataaagagaggagacttctcttttgatgaagtagatctcattttgaggcttcataagctgttaggcaacagatggtcacttattgctggtagacttcctggaaggacggcaaacgatgtcaaaaactactggaacagccatcttcgcaagaagttaattgctcctcatgatcaaaaggagagcaagcaaaaagcaaagaagatcaccatattcagacctcggcctcgaaccttctcaaagacaaatacttgtgttaaaagtaacacaaatactgtagataaggatattgaaggcagcagcgaaataattagattcaacgataatttgaagccaacaactgaagaattgacggatgatggaattcaatggtgggccgatttactagctaacaattacaacaataatgggattgaggaagctgataattcatcaccaactttgttgcatgaggaaatgccacttctcagttgatctagaaataacagagggcgcgcgagcggtggctactgatcgcctatgagttctgtgattctacttgtaatttcagaagtgttttcagtgtcttgttttctggaagtccgtctggtttttagtaacttttagctcaaaaatgtgtctgtacgatggtatttgtatgtttgtgggtcttttacatatacgcttgtaatcgatcaatgtagaatgctgtgtgccttttccgtcaacagcttatttagtgtttactctgtatacgtatatctaatatatagtactgattctttcatctggtgatttgttttcctaaagagattattatcatagctttaattgaatgatacaaagaggtgttgcctggcttcaccagagcagaaattttcattgatatagggtacaaatgtcattcacataatgttaagagataagtttttcaatgtcctcaagagcccaccaagagtttcttccgggaattgcttaaattatcttaaatttaaattgtaaaac

SEQ ID NO: 61 - DNA, 3701 bp, Artificial Sequence
  comprises plant native sequences only
cccgggaaactaataagaacaagcaatataagagaattcgtaaaaaactttctagttcttgaacatctacccatgtgaattctcttttatttttgtacactataattaaattaacatggctaaaccaattatgccaactgaataaattatcaatattgataaacttcaggtttacaccatgacgtgtgcaattatgaataaactccaagtttattatgatatgagtttttatatcaataaacttctactttactgtgacattcttttgtttgtgtagtacaaattggagaataaagcgtgtaacttttcacatacatattaccccgctataagttgtagtaatagaagatattaaatctttcctttctttatagtctcaatataaccaatcgcttttgcgaatactttagaaactaaataagtttctttgagacttactacaacataatgccttattgataatcaattttgttccttcaaaatagtaataattggctcttccagagctctcaattaattttgtactaccacatattcatcaacatccatatggtgaatatctcttttaaagagaaagttataccattatggttatggtcaaaattatatgcaatatttgtttcttgcattaccgttgccttttagtaatcacattgccaaaatattttggcctacaataagtacgtgaccaatgaccatttatgccataatgacattattttcttattttctctcaaacctccttcaagagatgagtgtggtatatactactagcacgctcatattcttccaaaaatgaatatgtattcataaatcacatattgtcacattcacatcatgaatggaccataatcatctatatgtgctttacaaaatctcatgtcaaatcgatgataaatattactttcacatagtgaatgattattttgagaatacttattattctcattaccacaatgaaaatgattataatttcgtctattgtcacatccacatccattgatacattcatggtaataattttatcttctttcagacgtatcatatattgctatcacattctcgtaagggaatgagaataaagcaaattcaatgggacgagtttccactttttgtgctcacaatcatacatgaatttgatcatggcaatacatagaaattttatcacttttggtggttataatttcttacaaactctattagagttataataaaaatttattgtctttgcttgtatttaaaatcaaattataaaattttaaaaattcaaaagagaaaaataaagtaaaatacttactttaaatccagaatttaatcacgaaggaagttcatggaataattgacgatcattatgctcaatcccaaagcttctactcaattggttacagtctcgtgccgataacgtgttataaaacaataaaagaagaacaatattgcagagaaagagagagagggaattcttattgaattttaggatgaattacaatggaataggacccctctatttatagggaaagagtgacttagccaccaagtaaaatccctaaaatctctctaaaatatagacattcaccttaaataaaactctatttataacaaaaacaaaattgttctagacgagaatcattttcactttttaatgtttttcttctactcctttagtttttccttaaaccaaaataaaaaaaaagtctatatttttctatcctttttcttctctagttttaatacattccataaaatttgtggtgaaattgtactttctccttttttttcctctttagtttcatagaaattaaacaataaaacgaaaacatcaaaatatatcaacaaatagtaaatttcattacatttatttttttgctcaaagtgctcttttgttgaatactcaaagtatatagtatattacagttctaatcaggaattattcactgaaatattgactgattttaggttcgtgtgatcgattaaatacctcttgaaccactacaaatttaacgaattaataacttttacctaacattttgttacccatgtattaatttgaatttatactattacttcctatttatgagtaatataacataatttctgtgtaaaggacagaaaatacagaatttgattaattcaaaattaattatacttcaaaaaatatcacaaggatatcaaaatttatcaaataaaggagcaacgtcattttcggctctcccacacaattcaaaataattcaaaacagaaccggctagacctaacctaaccaaaccatggttaatacaaatctaaatcaccgaaaaacaatcttaaccatagttaataacccgtattaattaacccgatatccatttcgccttgcccttattcattctcctataaaacagaggcccttcagtatagcgaagactcacaattcgaatttcgaaaactcatctctttctgttttaacggcgtcttgataaacgccgctccttctctcctcctctttgaaatttgaatttttagggtttcgtgaaactcgagaacaatgaatatttgtactaataagtcgtcgtcaggagtgaagaaaggtgcatggactgaagaagaagatgttctattgaaaaaatgcatcgagaaatatggagaaggaaagtggcatcaagttcctcttagagctggtttgaatagatgcagaaagagctgcagattaaggtggctaaattatctaaggccacatataaagagaggagacttctcttttgatgaagtagatctcattttgaggcttcataagctgttaggcaacagatggtcacttattgctggtagacttcctggaaggacggcaaacgatgtcaaaaactactggaacagccatcttcgcaagaagttaattgctcctcatgatcaaaaggagagcaagcaaaaagcaaagaagatcaccatattcagacctcggcctcgaaccttctcaaagacaaatacttgtgttaaaagtaacacaaatactgtagataaggatattgaaggcagcagcgaaataattagattcaacgataatttgaagccaacaactgaagaattgacggatgatggaattcaatggtgggccgatttactagctaacaattacaacaataatgggattgaggaagctgataattcatcaccaactttgttgcatgaggaaatgccacttctcagttgatctagaaataacagagggcgcgcgagcggtggctactgatcgcctatgagttctgtgattctacttgtaatttcagaagtgttttcagtgtcttgttttctggaagtccgtctggtttttagtaacttttagctcaaaaatgtgtctgtacgatggtatttgtatgtttgtgggtcttttacatatacgcttgtaatcgatcaatgtagaatgctgtgtgccttttccgtcaacagcttatttagtgtttactctgtatacgtatatctaatatatagtactgattctttcatctggtgatttgttttcctaaagagattattatcatagctttaattgaatgatacaaagaggtgttgcctggcttcaccagagcagaaattttcattgatatagggtacaaatgtcattcacataatgttaagagataagtttttcaatgtcctcaagagcccaccaagagtttcttccgggaattgcttaaattatcttaaatttaaattgtacccgtttaaac

SEQ ID NO: 62 - DNA, 6230 bp, Artificial Sequence
  comprises plant native sequences only
cccgggttagtattcaaaccgaataaatcaaagttaccaaaccgaataaatcgaaaccgaaaggagaaaccgcaccataccgaatttaattaggtacgatattgatattgtattttaaaaaatcgaataccaaaaataccgaattaaaatatctaaatatcgtacagtaccgaccgataaatactctataagcatcatcatgtcaccattcctgcttggaaatagatgtaataatgtaattcaaggtgaagatcattgaaaatgagatatttggactcttagataattgtgcaactgatatttttatttactttttttctttcatccaataattgcgttacattaaaaatgagatatttggattaatattcttctccttgaccacaaagcaaggaaagcctaaggaccgatagtaaagttgtattcgtgtggttgcgtgttagttttgagcggcaaaataaattatgttaaggtaaattatttttggaacaataataaaattatttctgtataatatataaatcatatatttgaaccgtagaattatcagttaatacttgtatatgaggaggctaactacgttagagcgctaacgagaatacttcatataccgtattttttacgataataataatgtaatgtgaaattgctatccaaaaggcacctaattttgtccaccgttcaaaggaaaggacaaggaagtagtagcgtgtaggtttggtgctgtacaaaataagcaagacacgtgttgccttattataggataatccataaggcaatttcgtcttaagtcggccattgcacctttaaaaggagcctctttgttcccaaaatcttcatcctttgatttctctattctcaatatctcctcaatttttctctagtcttcaaacacttctcaaggtacattaacttcttctttctttttgttcctcttattttatgctacttttatttaatttcgatctatatttttaggatctaaatactcatttttgatttgtttaatcgctctgtatatatgcaccaagttgaaatttttgtaagtttattttgttcggtctatattttaagatctgaaataccctttactgagaaaaaaaaaactcaaccttgattttgttgtacctggttgaatttgttattgttgtgtatacagttaaaaaactcaagtcttgattttattgtttcccttttgtagtttgtatatacatagagctgaattggtgttctaattttggttgatttttatgtatacagtataaaatcgatcttagttttgttcattgatttgtatttgcacaaagttggaattttgcgtttgttattttgatgattgaaaccttttctgtatatacagctcgagatgaatatttgtactaataagtcgtcgtcaggagtgaagaaaggtgcatggactgaagaagaagatgttctattgaaaaaatgcatcgagaaatatggagaaggaaagtggcatcaagttcctcttagagctggtttgaatagatgcagaaagagctgcagattaaggtggctaaattatctaaggccacatataaagagaggagacttctcttttgatgaagtagatctcattttgaggcttcataagctgttaggcaacagatggtcacttattgctggtagacttcctggaaggacggcaaacgatgtcaaaaactactggaacagccatcttcgcaagaagttaattgctcctcatgatcaaaaggagagcaagcaaaaagcaaagaagatcaccatattcagacctcggcctcgaaccttctcaaagacaaatacttgtgttaaaagtaacacaaatactgtagataaggatattgaaggcagcagcgaaataattagattcaacgataatttgaagccaacaactgaagaattgacggatgatggaattcaatggtgggccgatttactagctaacaattacaacaataatgggattgaggaagctgataattcatcaccaactttgttgcatgaggaaatgccacttctcagttgatctagaaataacagagggcgcgcgagcggtggctactgatcgcctatgagttctgtgattctacttgtaatttcagaagtgttttcagtgtcttgttttctggaagtccgtctggtttttagtaacttttagctcaaaaatgtgtctgtacgatggtatttgtatgtttgtgggtcttttacatatacgcttgtaatcgatcaatgtagaatgctgtgtgccttttccgtcaacagcttatttagtgtttactctgtatacgtatatctaatatatagtactgattctttcatctggtgatttgttttcctaaagagattattatcatagctttaattgaatgatacaaagaggtgttgcctggcttcaccagagcagaaattttcattgatatagggtacaaatgtcattcacataatgttaagagataagtttttcaatgtcctcaagagcccaccaagagtttcttccgggaattgcttaaattatcttaaatttaaattgtaaaactaataagaacaagcaatataagagaattcgtaaaaaactttctagttcttgaacatctacccatgtgaattctcttttatttttgtacactataattaaattaacatggctaaaccaattatgccaactgaataaattatcaatattgataaacttcaggtttacaccatgacgtgtgcaattatgaataaactccaagtttattatgatatgagtttttatatcaataaacttctactttactgtgacattcttttgtttgtgtagtacaaattggagaataaagcgtgtaacttttcacatacatattaccccgctataagttgtagtaatagaagatattaaatctttcctttctttatagtctcaatataaccaatcgcttttgcgaatactttagaaactaaataagtttctttgagacttactacaacataatgccttattgataatcaattttgttccttcaaaatagtaataattggctcttccagagctctcaattaattttgtactaccacatattcatcaacatccatatggtgaatatctcttttaaagagaaagttataccattatggttatggtcaaaattatatgcaatatttgtttcttgcattaccgttgccttttagtaatcacattgccaaaatattttggcctacaataagtacgtgaccaatgaccatttatgccataatgacattattttcttattttctctcaaacctccttcaagagatgagtgtggtatatactactagcacgctcatattcttccaaaaatgaatatgtattcataaatcacatattgtcacattcacatcatgaatggaccataatcatctatatgtgctttacaaaatctcatgtcaaatcgatgataaatattactttcacatagtgaatgattattttgagaatacttattattctcattaccacaatgaaaatgattataatttcgtctattgtcacatccacatccattgatacattcatggtaataattttatcttctttcagacgtatcatatattgctatcacattctcgtaagggaatgagaataaagcaaattcaatgggacgagtttccactttttgtgctcacaatcatacatgaatttgatcatggcaatacatagaaattttatcacttttggtggttataatttcttacaaactctattagagttataataaaaatttattgtctttgcttgtatttaaaatcaaattataaaattttaaaaattcaaaagagaaaaataaagtaaaatacttactttaaatccagaatttaatcacgaaggaagttcatggaataattgacgatcattatgctcaatcccaaagcttctactcaattggttacagtctcgtgccgataacgtgttataaaacaataaaagaagaacaatattgcagagaaagagagagagggaattcttattgaattttaggatgaattacaatggaataggacccctctatttatagggaaagagtgacttagccaccaagtaaaatccctaaaatctctctaaaatatagacattcaccttaaataaaactctatttataacaaaaacaaaattgttctagacgagaatcattttcactttttaatgtttttcttctactcctttagtttttccttaaaccaaaataaaaaaaaagtctatatttttctatcctttttcttctctagttttaatacattccataaaatttgtggtgaaattgtactttctccttttttttcctctttagtttcatagaaattaaacaataaaacgaaaacatcaaaatatatcaacaaatagtaaatttcattacatttatttttttgctcaaagtgctcttttgttgaatactcaaagtatatagtatattacagttctaatcaggaattattcactgaaatattgactgattttaggttcgtgtgatcgattaaatacctcttgaaccactacaaatttaacgaattaataacttttacctaacattttgttacccatgtattaatttgaatttatactattacttcctatttatgagtaatataacataatttctgtgtaaaggacagaaaatacagaatttgattaattcaaaattaattatacttcaaaaaatatcacaaggatatcaaaatttatcaaataaaggagcaacgtcattttcggctctcccacacaattcaaaataattcaaaacagaaccggctagacctaacctaaccaaaccatggttaatacaaatctaaatcaccgaaaaacaatcttaaccatagttaataacccgtattaattaacccgatatccatttcgccttgcccttattcattctcctataaaacagaggcccttcagtatagcgaagactcacaattcgaatttcgaaaactcatctctttctgttttaacggcgtcttgataaacgccgctccttctctcctcctctttgaaatttgaatttttagggtttcgtgaaactcgagaacaatgaatatttgtactaataagtcgtcgtcaggagtgaagaaaggtgcatggactgaagaagaagatgttctattgaaaaaatgcatcgagaaatatggagaaggaaagtggcatcaagttcctcttagagctggtttgaatagatgcagaaagagctgcagattaaggtggctaaattatctaaggccacatataaagagaggagacttctcttttgatgaagtagatctcattttgaggcttcataagctgttaggcaacagatggtcacttattgctggtagacttcctggaaggacggcaaacgatgtcaaaaactactggaacagccatcttcgcaagaagttaattgctcctcatgatcaaaaggagagcaagcaaaaagcaaagaagatcaccatattcagacctcggcctcgaaccttctcaaagacaaatacttgtgttaaaagtaacacaaatactgtagataaggatattgaaggcagcagcgaaataattagattcaacgataatttgaagccaacaactgaagaattgacggatgatggaattcaatggtgggccgatttactagctaacaattacaacaataatgggattgaggaagctgataattcatcaccaactttgttgcatgaggaaatgccacttctcagttgatctagaaataacagagggcgcgcgagcggtggctactgatcgcctatgagttctgtgattctacttgtaatttcagaagtgttttcagtgtcttgttttctggaagtccgtctggtttttagtaacttttagctcaaaaatgtgtctgtacgatggtatttgtatgtttgtgggtcttttacatatacgcttgtaatcgatcaatgtagaatgctgtgtgccttttccgtcaacagcttatttagtgtttactctgtatacgtatatctaatatatagtactgattctttcatctggtgatttgttttcctaaagagattattatcatagctttaattgaatgatacaaagaggtgttgcctggcttcaccagagcagaaattttcattgatatagggtacaaatgtcattcacataatgttaagagataagtttttcaatgtcctcaagagcccaccaagagtttcttccgggaattgcttaaattatcttaaatttaaattgtacccgtttaaac

SEQ ID NO: 63 - DNA, 7583 bp, Artificial Sequence
  comprises plant native sequences only
cccgggttagtattcaaaccgaataaatcaaagttaccaaaccgaataaatcgaaaccgaaaggagaaaccgcaccataccgaatttaattaggtacgatattgatattgtattttaaaaaatcgaataccaaaaataccgaattaaaatatctaaatatcgtacagtaccgaccgataaatactctataagcatcatcatgtcaccattcctgcttggaaatagatgtaataatgtaattcaaggtgaagatcattgaaaatgagatatttggactcttagataattgtgcaactgatatttttatttactttttttctttcatccaataattgcgttacattaaaaatgagatatttggattaatattcttctccttgaccacaaagcaaggaaagcctaaggaccgatagtaaagttgtattcgtgtggttgcgtgttagttttgagcggcaaaataaattatgttaaggtaaattatttttggaacaataataaaattatttctgtataatatataaatcatatatttgaaccgtagaattatcagttaatacttgtatatgaggaggctaactacgttagagcgctaacgagaatacttcatataccgtattttttacgataataataatgtaatgtgaaattgctatccaaaaggcacctaattttgtccaccgttcaaaggaaaggacaaggaagtagtagcgtgtaggtttggtgctgtacaaaataagcaagacacgtgttgccttattataggataatccataaggcaatttcgtcttaagtcggccattgcacctttaaaaggagcctctttgttcccaaaatcttcatcctttgatttctctattctcaatatctcctcaatttttctctagtcttcaaacacttctcaaggtacattaacttcttctttctttttgttcctcttattttatgctacttttatttaatttcgatctatatttttaggatctaaatactcatttttgatttgtttaatcgctctgtatatatgcaccaagttgaaatttttgtaagtttattttgttcggtctatattttaagatctgaaataccctttactgagaaaaaaaaaactcaaccttgattttgttgtacctggttgaatttgttattgttgtgtatacagttaaaaaactcaagtcttgattttattgtttcccttttgtagtttgtatatacatagagctgaattggtgttctaattttggttgatttttatgtatacagtataaaatcgatcttagttttgttcattgatttgtatttgcacaaagttggaattttgcgtttgttattttgatgattgaaaccttttctgtatatacagctcgagatgacggagataccgcctaacagccagatgaaaaccatgttgcagaaggcagtgcaatcggttcaatggacatatactcttttctggcaattatgtccccaacaaggggcgttagtgtggagagatggatattacaatggggctataaagactagaaagacagtgcagccaatggaagttagcgctgaggaagcttctcttcacagaagccaacagcttagagaactttacgaatcactttccgccggcgagtcaaatcagccagcgagaaggccgtcggcagctttgtcaccggaggacttgacggagtccgagtggttttatctcatgtgtgtttctttctcttttcctcctggcatcggattacctggcaaggcttattcgaagaaacatcacatatggatcatgggcgcaaacgaggttgatagcaaagtcttctgtagagctattcttgccaagagcgcccgcatacagacggtcgttggtattcctctcttggatggtgtactggaactgggaactacagaaagggttcaagaagagattggattcataaaccatgtaaagagctttttcactgagcaacaacaacctcagctaccaaagccagccttatctgagcactccacttccaatcccaccaccttttccgagccacatttttactccggcaatacttcgccatctgctaatgttgatattgcgcatcaagatggcggagctgccggcgaagaagatgaggaggaggaagaagaagaagatgatgatgaagccgagttggactcggatagtatagcgattcaaagcgcggctaatcctattgccgttgaggctagtgaactcatgcagcttgatgtgtccgaggctatacagctcggctcgcccgatgatgactctgataatatggactctgattttcatttggttggcgctggaaacacggctcatgactaccagcgccaagctgactctttcaaagccgagaccgccattagctggccgcacttccaagaccttcaacaattaccaggtggctctagttatgatgaattatcacaagaagacacacactattctcaaacagtgtcaaccattctcgaacaccgaagctccaaattttcctctacaacaatgggctgtatttctcatgactcggcccaatctgccttcacattgtgccctagcaccaccgtctgcagcccgaatcccgcccactgccgccacgacgactcacttgtcgacggtggcggcgcctcccagtggctgctcaaaagcatactcttcactgtcccatttcttcacactaaataccaatctgaagcttctccaaagtcacgtgacgtcgccactgttgattcctccagtactgcttctcgctttcgcaaaggctgtagtataacgtcgcaagaagagccaagtggaaaccatgtacttgcagaacgacgtcgtagagagaagctaaatgagcgttttatcatattaaggtctcttgtaccttttgtaacgaaaatggacaaagcctccattttgggtgacaccatagagtatgtcaagcagttacgtaagaaagttcaggatcttgaagctcgtgctcgcgacacggagcactccagagatgcagataaaaaaggtggcacagctacagtgaaggtgttgcaaggaaggggtaagaggagaatgaatacggtagatggaagtgttggtggagggcaggcaacgataacggcgtccccaccgtcaacgacggaaaatgaggaggttgtgcaagtacaagtatcaattatcgaaagcgatgcattggtggagctccggtgtccgtacaaagaggggttgctgttaaatgtaatgcagatgctaagggaactcaaagtggaagttgtagccattcaatcagctcttaataatggcgtcttcttggctgagttaagagctaaggtaaaagagaatatatgtggaaggaaagcaagcattttggaagtaaaaaggtcaatacatcagataatccctagagattaatctagaaataacagagggcgcgcgagcggtggctactgatcgcctatgagttctgtgattctacttgtaatttcagaagtgttttcagtgtcttgttttctggaagtccgtctggtttttagtaacttttagctcaaaaatgtgtctgtacgatggtatttgtatgtttgtgggtcttttacatatacgcttgtaatcgatcaatgtagaatgctgtgtgccttttccgtcaacagcttatttagtgtttactctgtatacgtatatctaatatatagtactgattctttcatctggtgatttgttttcctaaagagattattatcatagctttaattgaatgatacaaagaggtgttgcctggcttcaccagagcagaaattttcattgatatagggtacaaatgtcattcacataatgttaagagataagtttttcaatgtcctcaagagcccaccaagagtttcttccgggaattgcttaaattatcttaaatttaaattgtaaaactaataagaacaagcaatataagagaattcgtaaaaaactttctagttcttgaacatctacccatgtgaattctcttttatttttgtacactataattaaattaacatggctaaaccaattatgccaactgaataaattatcaatattgataaacttcaggtttacaccatgacgtgtgcaattatgaataaactccaagtttattatgatatgagtttttatatcaataaacttctactttactgtgacattcttttgtttgtgtagtacaaattggagaataaagcgtgtaacttttcacatacatattaccccgctataagttgtagtaatagaagatattaaatctttcctttctttatagtctcaatataaccaatcgcttttgcgaatactttagaaactaaataagtttctttgagacttactacaacataatgccttattgataatcaattttgttccttcaaaatagtaataattggctcttccagagctctcaattaattttgtactaccacatattcatcaacatccatatggtgaatatctcttttaaagagaaagttataccattatggttatggtcaaaattatatgcaatatttgtttcttgcattaccgttgccttttagtaatcacattgccaaaatattttggcctacaataagtacgtgaccaatgaccatttatgccataatgacattattttcttattttctctcaaacctccttcaagagatgagtgtggtatatactactagcacgctcatattcttccaaaaatgaatatgtattcataaatcacatattgtcacattcacatcatgaatggaccataatcatctatatgtgctttacaaaatctcatgtcaaatcgatgataaatattactttcacatagtgaatgattattttgagaatacttattattctcattaccacaatgaaaatgattataatttcgtctattgtcacatccacatccattgatacattcatggtaataattttatcttctttcagacgtatcatatattgctatcacattctcgtaagggaatgagaataaagcaaattcaatgggacgagtttccactttttgtgctcacaatcatacatgaatttgatcatggcaatacatagaaattttatcacttttggtggttataatttcttacaaactctattagagttataataaaaatttattgtctttgcttgtatttaaaatcaaattataaaattttaaaaattcaaaagagaaaaataaagtaaaatacttactttaaatccagaatttaatcacgaaggaagttcatggaataattgacgatcattatgctcaatcccaaagcttctactcaattggttacagtctcgtgccgataacgtgttataaaacaataaaagaagaacaatattgcagagaaagagagagagggaattcttattgaattttaggatgaattacaatggaataggacccctctatttatagggaaagagtgacttagccaccaagtaaaatccctaaaatctctctaaaatatagacattcaccttaaataaaactctatttataacaaaaacaaaattgttctagacgagaatcattttcactttttaatgtttttcttctactcctttagtttttccttaaaccaaaataaaaaaaaagtctatatttttctatcctttttcttctctagttttaatacattccataaaatttgtggtgaaattgtactttctccttttttttcctctttagtttcatagaaattaaacaataaaacgaaaacatcaaaatatatcaacaaatagtaaatttcattacatttatttttttgctcaaagtgctcttttgttgaatactcaaagtatatagtatattacagttctaatcaggaattattcactgaaatattgactgattttaggttcgtgtgatcgattaaatacctcttgaaccactacaaatttaacgaattaataacttttacctaacattttgttacccatgtattaatttgaatttatactattacttcctatttatgagtaatataacataatttctgtgtaaaggacagaaaatacagaatttgattaattcaaaattaattatacttcaaaaaatatcacaaggatatcaaaatttatcaaataaaggagcaacgtcattttcggctctcccacacaattcaaaataattcaaaacagaaccggctagacctaacctaaccaaaccatggttaatacaaatctaaatcaccgaaaaacaatcttaaccatagttaataacccgtattaattaacccgatatccatttcgccttgcccttattcattctcctataaaacagaggcccttcagtatagcgaagactcacaattcgaatttcgaaaactcatctctttctgttttaacggcgtcttgataaacgccgctccttctctcctcctctttgaaatttgaatttttagggtttcgtgaaactcgagaacaatgaatatttgtactaataagtcgtcgtcaggagtgaagaaaggtgcatggactgaagaagaagatgttctattgaaaaaatgcatcgagaaatatggagaaggaaagtggcatcaagttcctcttagagctggtttgaatagatgcagaaagagctgcagattaaggtggctaaattatctaaggccacatataaagagaggagacttctcttttgatgaagtagatctcattttgaggcttcataagctgttaggcaacagatggtcacttattgctggtagacttcctggaaggacggcaaacgatgtcaaaaactactggaacagccatcttcgcaagaagttaattgctcctcatgatcaaaaggagagcaagcaaaaagcaaagaagatcaccatattcagacctcggcctcgaaccttctcaaagacaaatacttgtgttaaaagtaacacaaatactgtagataaggatattgaaggcagcagcgaaataattagattcaacgataatttgaagccaacaactgaagaattgacggatgatggaattcaatggtgggccgatttactagctaacaattacaacaataatgggattgaggaagctgataattcatcaccaactttgttgcatgaggaaatgccacttctcagttgatctagaaataacagagggcgcgcgagcggtggctactgatcgcctatgagttctgtgattctacttgtaatttcagaagtgttttcagtgtcttgttttctggaagtccgtctggtttttagtaacttttagctcaaaaatgtgtctgtacgatggtatttgtatgtttgtgggtcttttacatatacgcttgtaatcgatcaatgtagaatgctgtgtgccttttccgtcaacagcttatttagtgtttactctgtatacgtatatctaatatatagtactgattctttcatctggtgatttgttttcctaaagagattattatcatagctttaattgaatgatacaaagaggtgttgcctggcttcaccagagcagaaattttcattgatatagggtacaaatgtcattcacataatgttaagagataagtttttcaatgtcctcaagagcccaccaagagtttcttccgggaattgcttaaattatcttaaatttaaattgtacccgtttaaac

SEQ ID NO: 64 - protein, 299 aa, Nicotiana
MGRKPCCAKEGLRKGPWSSKEDLLLTNYIKENGEGQWRSLPKNAGLLRCGKSCRLRWMNYLRPGIKRGNFSQDEEDLILRLHSLLGNRWSLIAGRLPGRTDNEIKNYWNTHLIKKLKSAGIEPKPHKKFSKCSKKESRKGPQQEKSRKKQGKKSNNKNNEGQIVQVEKIQVFTPKPIRISSEVLSRNNSFENVTLSTNCSSNSNFEEADVDIKETELKLEEVSFFPRDLDFGKLLEGDANLDEFLIQESSYISNKYSVPMNESMLEKVYEEYLLLLSENCYLQDDHQKEQNFPVNVSDQ

SEQ ID NO: 65 - protein, 240 aa, Nicotiana
MNYLRPGIKRGNFTQDEEDLIVRLHSLLGNRWSLIAGRLPGRTDNEIKNYWNTHLIKKLKSAGIERKPHKNFSKCSKKESRKGPQQEKSRKKQGKKSNNKNNEGQIVQVEKIQVFTPKPIRISSEVLSRNNSFENVTLSTTCSSNSNFEEADVENKEKEVKLEEVSFFPRDLNFGKLLEGDENLDEFLIQENSCISNKHSMLMNESMLEKVYEEYLLLLSENCYLQDDHQKEQNFPCKCL

SEQ ID NO: 66 - DNA, 900 bp, Nicotiana
atgggaagaaaaccatgttgtgcaaaagagggattgcgaaaaggtccttggtcttctaaagaagatttgttacttactaattatatcaaggaaaatggtgaaggacaatggagatctttgcctaagaatgctgggttgcttaggtgtggaaaaagttgcagactaagatggatgaactatttaagaccagggattaaaagaggaaacttcagtcaagatgaagaagatcttatattgagactacattctcttttgggtaatcgttggtcactaattgctgggagattaccaggtcgaacagataatgaaatcaagaattattggaacacccatttaatcaagaagctcaaaagtgctggaattgaaccaaaaccccacaaaaaattctccaaatgttccaaaaaggaatcaagaaaaggaccccaacaagagaaatcaagaaaaaaacaaggtaaaaagagcaacaacaaaaacaatgagggtcaaattgtacaagttgagaaaattcaagtgtttaccccaaaacccatcaggatttcttctgaggtactttcaaggaacaatagttttgaaaatgttacattgagtactaattgttcctcaaatagtaattttgaagaagctgatgttgacatcaaggaaactgagttgaaattagaagaagtttcattctttccaagggacttagattttggcaaattacttgaaggggatgcaaatttagatgaatttcttattcaagaaagcagctacatttcaaacaaatattcagtgccaatgaatgagagcatgttggagaaagtgtatgaagaatatcttttacttctttctgaaaattgttaccttcaagatgatcatcaaaaggagcaaaatttccctgtaaatgtctctgatcagtga

SEQ ID NO: 67 - DNA, 723 bp, Nicotiana
atgaactatttaagaccagggattaaaagaggaaacttcactcaagatgaagaagatcttatagtgagactacattctcttttgggtaatcgttggtcactaattgctggaagattaccaggtcgaacagataatgaaatcaaaaattattggaacacccatttaatcaagaagctcaaaagtgctggaattgaacgaaaaccccacaaaaatttctccaaatgttccaaaaaggaatcaagaaaaggaccccaacaagagaaatcaagaaaaaaacaaggcaaaaagagcaacaacaaaaacaatgagggtcaaattgtacaagttgagaaaattcaagtgtttaccccaaaacccatcaggatttcttctgaggtactttcaaggaacaatagttttgaaaatgttacattgagtactacttgttcctcaaatagtaattttgaagaagctgatgttgaaaacaaggaaaaagaggtgaaattagaagaagtttcattctttccaagggacttaaattttggtaaattacttgaaggggatgaaaatttagatgaatttcttattcaagaaaacagctgcatttcaaacaaacattcaatgctaatgaatgagagcatgttggagaaagtatatgaagaatatcttttacttctttctgaaaattgttaccttcaagatgatcatcaaaaggagcaaaatttcccctgtaaatgtctctga

SEQ ID NO: 68 - protein, 318 aa, Nicotiana
MEAQLLKLPSPSLTSTNSSKHSTLLPRQKWSNFCKFQLPNSTSTITIRPLQASATSLGLGPKKRIDETESYTLDGIRNSLIRQEDSIIFSLVERAQYCYNAETYDPDVFLMDGFHGSLVEYIVKETEKLHAKVGRYKSPDEHPFFPKELPEPMLPPMQFPKVLHSVADSININVKIWEMYFKNLLPRLVKEGDDGNFGSTAVCDTICLQALSKRIHYGKFVAEAKFRASPDVYKAAIRAQDRNGLMDLLTYPTVEEAITRRVEMKTRTYGQEFNINGPENGGDPVYKIKPSLVAELYGDWIMPLTKEVQVEYLLRRLD

SEQ ID NO: 69 - protein, 262 aa, Nicotiana
MALISGDANNKLSLDSIRDSLIRQEDTIIFNLIERIKYPINSTLYKEPSSSSSWNISGSLFHYLFQETEALQSKVGRYLSPEENPFFPDNLPASIIPPSKCTPVLHPAAESVNVNEKILDVYIKQLLPLFCITDQADEGNFATIASCDIQLLQALSRRIHYGKFVAEIKFRDCTDQYKPLILAKDRDALMKLLTFEAVEEMVKKRVAKKALTFGQQVTLNIDDSSKEVKCKVDPSLVSRLYDEWIMPLTKLVEVEYLLRRLD

SEQ ID NO: 70 - protein, 257 aa, Nicotiana
MASDNNKLSLDSIRDSLIRQEDTIIFNLIERIKYPITPTLYKEASSSSWNISGSLFHYLFQETEALHSKVGRYLSAEENPFFPDKLPASIIPPSKCTPVLHPAAECVNVNEKILDVYKKQLLPLFCTDQADDEENFATTASCDIQLLQALSRRIHYGKFVAKVKFRDCTDQYKPLILAKDRDALMKLLTFEAVEEVVKKRVAKKAFVFGQQVTLNIDDNTKEAKYKVDPSLVSRLYDEWIMPLTKLVEVEYLLRRLD

SEQ ID NO: 71 - DNA, 957 bp, Nicotiana
atggaagcccaattgttaaaactcccttctccttccttaacaagtaccaattcttcaaaacacagtacccttttaccccgtcaaaaatggtcaaatttttgtaagtttcaattacccaattcaactagtaccattactattcgtccccttcaagcttctgctacttctcttggacttgggccaaagaagagaatagatgagacggagagttacactcttgatggtataaggaactctttaattcgacaagaagatagcataatattcagccttgtggagagagctcagtactgttacaatgcggagacatatgatcctgatgtttttttgatggatgggtttcatggctctttggttgaatatattgtcaaagaaactgaaaagcttcatgctaaggttggaagatataaaagccctgatgagcacccattcttcccaaaagaattacccgagccaatgttgccacccatgcagttcccaaaggttctgcattcagttgctgattcaataaatatcaatgtcaaaatatgggaaatgtatttcaagaatctcctcccaagattagtaaaggaaggcgacgatggtaattttggatctacagcagtttgtgacactatttgcttgcaggccctgtcgaagagaattcattatgggaaatttgtcgctgaagcaaaatttcgagcctcaccagatgtctataaggctgccataagagcacaagacagaaacggactgatggatttgttaacctaccctactgttgaagaggctatcacgaggagggtagaaatgaaaaccagaacttacggacaagaatttaacatcaatggaccggaaaatggaggtgacccagtgtacaaaataaaaccaagcctagttgctgaattgtacggcgactggatcatgccattgacaaaggaagttcaagttgagtatctcctgagaagactggattag

SEQ ID NO: 72 - DNA, 789 bp, Nicotiana
atggctttaattagtggtgatgctaataataaactgagtcttgattcaataagggatagtttaataagacaagaagacaccatcattttcaaccttatagagagaatcaaatacccaataaattccaccttgtacaaagaaccttcttcttcttcttcttggaatatttcagggtccttgttccactatttgtttcaagaaacagaagctcttcaatctaaggttggtagatacctatcaccagaagaaaatcctttcttcccagataacttgcctgcctcaatcataccacctagcaaatgcacaccagttttgcatcctgcagcagaatctgtcaacgtaaatgagaagatattggatgtttatataaagcagttgcttccactattttgtattactgatcaggctgatgaaggaaactttgcaactattgcttcctgtgatattcagttattgcaggcactctctagaaggattcattatggaaaatttgttgctgagattaaattcagggattgtactgatcaatataaaccacttattcttgctaaggatagggatgctctaatgaagctattgacatttgaagcagttgaagagatggtaaagaagagagttgcaaagaaagccttgacgtttgggcaacaagtgaccctaaatattgatgatagctccaaagaagtaaagtgcaaggttgatccatcgctagtttcgcgcttatatgatgaatggattatgcctttgacaaaacttgttgaagttgagtaccttctacgacgtctcgattag

SEQ ID NO: 73 - DNA, 774 bp, Nicotiana
atggcatcggataataataaactgagtcttgattcaataagggatagtttaattagacaagaagacaccatcattttcaaccttatagagagaatcaaatacccaataactcccaccttgtacaaagaagcttcttcttcttcttggaatatttcagggtcattgttccactacttgtttcaagaaacagaagctcttcattctaaggttggtagatacctatcagcagaggaaaatcctttcttcccagataagttgcctgcctcaatcataccacctagcaaatgcacaccagttttgcatcctgcagcagaatgtgtgaacgtaaatgagaagatattggatgtttataaaaagcagttgcttccactattttgtactgatcaggctgacgatgaagaaaactttgcaactactgcttcctgtgatattcagttattgcaggcactctctagaaggattcattatgggaaatttgttgctaaggttaaattcagggattgtactgatcaatataaaccacttattcttgctaaggatagggatgctctaatgaagctattgacatttgaagcagttgaagaggtggtaaaaaagagagttgcaaagaaagcatttgtgtttgggcaacaagtgaccctaaatattgatgataacaccaaagaagcaaagtacaaggttgatccatcactggtttcgcgcttatatgatgaatggataatgcctttgacaaaacttgtcgaagttgagtaccttctacgccgtcttgattag